European Patent Application EP 4 737 579 A2, published May 6, 2026. Title: GLUCOAMYLASE ENGINEERED YEAST AND FERMENTATION METHODS. Applicant: CARGILL, INCORPORATED. Application WO PCT/US2019/019805, filed February 27, 2019. The sequence listing filed with the application follows.

SEQUENCE LISTING (29 sequences)

SEQ ID NO: 1 - protein, 605 aa, Rhizopus microsporus
MKLMNPSMKAYVFFILSYFSLLVSSAAVPTSAAVQVESYNYDGTTFSGRIFVKNIAYSKVVTVIYSDGSDNWNNNNNKVSAAYSEAISGSNYEYWTFSAKLSGIKQFYVKYEVSGSTYYDNNGTKNYQVQATSATSTTATATTTTATGTTTTSTGPTSTASVSFPTGNSTISSWIKNQEEISRFAMLRNINPPGSATGFIAASLSTAGPDYYYSWTRDSALTANVIAYEYNTTFTGNTTLLKYLKDYVTFSVKSQSVSTVCNCLGEPKFNADGSSFTGPWGRPQNDGPAERAVTFMLIADSYLTQTKDASYVTGTLKPAIFKDLDYVVSVWSNGCYDLWEEVNGVHFYTLMVMRKGLILGADFAARNGDSSRASTYKQTASTMESKISSFWSDSNNYVQVSQSVTAGVSKKGLDVSTLLAANIGSLPDGFFTPGSEKILATAVALENAFASLYPINSNLPSYLGNSIGRYPEDTYNGNGNSQGNPWFLAVNAYAELYYRAIKEWISNGKVTVSNISLPFFKKFDSSATSGKTYTAGTSDFNNLAQNIALGADRFLSTVKFHAYTNGSLSEEYDRSTGMSTGARDLTWSHASLITVAYAKAGSPAA

SEQ ID NO: 2 - DNA, 1818 bp, Rhizopus microsporus
  source 1..1818: mol_type = genomic DNA
atgaagctaatgaacccatctatgaaagcttatgtctttttcatcttatcatacttctctctcctagtttcatctgccgcagtgcctacatctgctgccgtccaagtggaaagttacaattacgatggcactaccttctccggccgtatcttcgtgaaaaacattgcttactcaaaagttgttacagtgatttactccgatggttctgataattggaacaacaataacaacaaagtttcagcagcgtactccgaagccattagtggatctaactacgaatactggactttctccgcaaagttgtctggtattaagcaattctacgtaaagtacgaagtttcaggttcaacatactacgataacaatggtactaaaaactaccaggtacaagccacaagcgctacaagtacaactgccacagctacaactacaactgctacagggacaacaactacatcaaccggtccaacatcaaccgcatctgtctcctttccaaccggtaacagtacaatatcatcatggatcaaaaaccaagaggaaatctcaagatttgcaatgttgagaaacatcaatccaccagggtcagcgactggtttcatcgccgcttcattgtccaccgctgggccagactactattactcttggactagagactctgcattgacagcaaacgttatagcttacgaatacaacacaaccttcactggtaacactaccttgttgaagtatcttaaagactacgtcacttttagtgttaagtctcaatctgtttctaccgtctgtaactgtttaggtgaaccaaagtttaatgcagatggctcatcatttactggtccatggggcagacctcaaaacgatggaccagcagaaagagcagtcacattcatgttgatcgctgactcatacttgacacaaactaaggatgcttcatacgtgactggaacactcaagccagccatattcaaagacctggattatgttgtttctgtgtggtctaatggttgctacgatttgtgggaggaagttaatggcgtacatttctacacactaatggttatgagaaagggactaattcttggggcagatttcgcagctagaaatggtgattcctcaagagcatctacctacaagcaaacagcatctacaatggaatcaaagatcagctctttctggtctgactctaacaactacgttcaagtttcacaatctgtgactgctggtgtaagtaaaaagggtttagatgtttctactctgttagctgcaaacattggttctttaccagatggcttctttacaccaggatcagaaaagattttggcaactgccgttgccttagagaatgcattcgcttccctttaccctattaactctaacttaccttcatatttgggtaattcaattggtagatatccagaggacacatacaacggaaacgggaattcacagggcaacccttggttcttagccgtaaacgcgtacgccgagttatactacagagccattaaggaatggatctcaaatggtaaggtaacagtctctaatatctctcttcctttctttaaaaagttcgattctagcgccactagcggcaagacctatacagccggaacaagtgatttcaataacctcgctcagaacatagctcttggagcagacagatttctgtcaactgttaaatttcacgcgtacacaaatggcagcttgtctgaagagtacgatcgttccaccgggatgagtactggtgctagagatctaacctggtcccatgcatctcttatcacagttgcatacgcaaaagctggatctcctgctgcgtaa

SEQ ID NO: 3 - DNA, 1818 bp, Rhizopus microsporus
  source 1..1818: mol_type = genomic DNA
atgaaacttatgaatccatctatgaaggcatacgttttctttatcttaagctacttctctttactcgttagctcagctgcggtgccaacctctgccgccgtacaagttgagtcatacaattatgacggtaccactttttcaggtagaatattcgtcaaaaacattgcctactcaaaggtcgtaacagttatctactccgatggatcagataactggaacaataacaacaacaaagtttctgcagcttactcagaagcaatttctgggtctaactacgaatactggacattctccgcaaagttatccggaattaaacagttttatgtcaaatacgaagtttctggttcaacatattacgacaacaacggtaccaaaaactaccaagtccaagcaacctcagcgacatctacaacagctactgcaaccacaactacagctactggcacaacaactacttctacaggtccaactagtactgcatccgtatcattccctaccggtaactcaacaatttcttcctggataaaaaatcaagaggaaatcagccgttttgctatgttgagaaatatcaatccacctgggtctgccacagggttcatagccgcatctctgtccacagccggcccagattactattactcttggactagagattcagcactaacagctaatgtgatcgcttacgaatacaacacaacattcactggaaacaccacccttcttaagtacttgaaagattacgttacattttctgtcaaaagccaatctgtatctaccgtttgtaactgtctgggagaaccaaagttcaacgctgatggtagttcttttacaggtccatggggcagaccacaaaacgacggaccagcagagagagctgttacttttatgttgattgctgacagctacttgactcaaactaaggacgcatcctacgttaccggtacattaaagccagcaatcttcaaagatcttgattacgtagtttctgtttggtctaacggttgctacgatttatgggaagaggttaatggtgttcatttctatactctcatggtcatgagaaagggtttgatcttaggtgccgacttcgctgctagaaatggtgactctagtagagcttcaacctacaagcaaactgcatcaacaatggaatcaaagatcagttctttttggtcagattctaacaactacgtccaagtttctcaatcagttaccgccggagtgtcaaaaaagggactagatgttagtacactattggcggccaacattggtagtctgcctgatggctttttcactccaggctccgaaaagatattggctacagcagtggcgttagaaaatgcattcgcatccttgtacccaattaactctaacctaccttcttacttgggtaactcaattggaagatatcctgaggatacatacaacggtaatggcaactctcaggggaatccatggttccttgccgtcaacgcatacgcagaactttactacagagctattaaggaatggattagtaatggcaaggtgacagtatccaatatctcactacctttcttcaaaaagtttgattcttccgccacttctggaaagacatacactgctggtacatcagatttcaataacttggctcagaacattgctttaggcgccgatagattcctgtctactgttaagttccacgcatacactaacgggagtctatcagaagagtacgatagatctaccggtatgagtactggggctcgtgatttaacatggtcccatgcttcattgatcacagtggcgtacgcaaaggccggtagtcctgcagcttag

SEQ ID NO: 4 - protein, 604 aa, Rhizopus delemar
MQLFNLPLKVSFFLVLSYFSLLVSAASIPSSASVQLDSYNYDGSTFSGKIYVKNIAYSKKVTVIYADGSDNWNNNGNTIAASYSAPISGSNYEYWTFSASINGIKEFYIKYEVSGKTYYDNNNSANYQVSTSKPTTTTATATTTTAPSTSTTTPPSSSEPATFPTGNSTISSWIKKQEGISRFAMLRNINPPGSATGFIAASLSTAGPDYYYAWTRDAALTSNVIVYEYNTTLSGNKTILNVLKDYVTFSVKTQSTSTVCNCLGEPKFNPDGSGYTGAWGRPQNDGPAERATTFILFADSYLTQTKDASYVTGTLKPAIFKDLDYVVNVWSNGCFDLWEEVNGVHFYTLMVMRKGLLLGADFAKRNGDSTRASTYSSTASTIANKISSFWVSSNNWIQVSQSVTGGVSKKGLDVSTLLAANLGSVDDGFFTPGSEKILATAVAVEDSFASLYPINKNLPSYLGNSIGRYPEDTYNGNGNSQGNPWFLAVTGYAELYYRAIKEWIGNGGVTVSSISLPFFKKFDSSATSGKKYTVGTSDFNNLAQNIALAADRFLSTVQLHAHNNGSLAEEFDRTTGLSTGARDLTWSHASLITASYAKAGAPAA

SEQ ID NO: 5 - DNA, 1815 bp, Rhizopus delemar
  source 1..1815: mol_type = genomic DNA
atgcagctgttcaacttgccattaaaggtttcattctttttggtcctatcatactttagtttgttggtgtcagccgcatctattccatcttcagcatctgtacaattagactcctacaattacgacggctctacattcagcggaaagatttacgtgaaaaatattgcgtacagcaaaaaagtaactgttatctatgccgacggatcagataactggaacaacaatggaaacactatcgctgccagttactctgcaccaatttcaggttctaactacgaatattggacattctcagcctccatcaatggcattaaggaattctacataaagtacgaagtttccggtaagacttactacgataacaacaattctgcaaactatcaagtatcaacatcaaaacctactaccaccaccgccacagctacaactacaactgcaccttcaacatctaccacaaccccaccatcttctagcgaaccagctacattcccaactggcaattctactatttctagttggatcaaaaaacaagagggtatttccagattcgcaatgttgagaaacataaatccaccaggatcagcaactggattcatcgcagcttctttgtccacagcggggccagattactactacgcatggaccagagatgctgctttgacaagtaacgttattgtttacgaatacaataccactttgtccggtaacaagactattcttaacgtcctaaaggattacgttacattctctgttaagactcagtctacatccacagtctgcaattgtttgggtgaaccaaagttcaacccagatggctctggatacacaggtgcctggggtcgtccacaaaacgatgggcctgccgagagagccactacatttatcctatttgctgactcataccttacacaaacaaaagatgcatcctacgtgactggaacattaaagcctgcaatcttcaaagacctggattacgttgtcaacgtgtggtctaacggctgtttcgatctatgggaagaggttaacggcgtgcacttctacactctaatggtcatgagaaagggtctgttgttaggtgcagattttgctaagagaaacggtgattctacacgtgcttctacctactcctcaacagcatcaactattgcgaacaagatttcttcattttgggtttcaagtaataactggatacaagtatctcaaagcgttacagggggtgtctcaaaaaagggtcttgatgtttctacattactggctgctaatcttgggtctgttgatgacggtttcttcacccctggttctgaaaagatcctcgctaccgccgtcgcggttgaggatagttttgcttcactctatcctataaacaaaaaccttccttcatacttaggaaacagtatcggtagatacccagaggatacatacaatggtaatggcaattcacagggaaatccatggttccttgctgttacagggtacgcagaactttactatagagctattaaggaatggatcggcaacggcggtgtgacagtttcctcaatctcattgccatttttcaaaaagtttgactccagcgcgacatctggtaaaaagtatactgtggggacttctgatttcaacaatttggctcaaaacattgccttagctgccgacagattcttatctaccgtacaactccatgcacataacaatggtagtttggcagaggaatttgatagaactacaggactctctacaggtgcgagagatttaacttggtcacatgcaagtttaattacagcctcttacgcaaaggctggtgctcctgctgcataa

SEQ ID NO: 6 - DNA, 1815 bp, Rhizopus delemar
  source 1..1815: mol_type = other DNA
atgcagttattcaacttaccacttaaggtatctttctttctagtcttatcttacttttcattgttagtatcagctgcctctataccaagttcagcatccgtacaactagattcatacaattacgacggttcaacattctcaggaaagatatacgtgaaaaatattgcttacagcaaaaaggttactgtgatttacgcagatgggtcagacaactggaataacaatggaaacacaattgctgcttcctattctgcccctatttctggatctaactacgaatactggactttttcagcgagtataaacggaattaaggaattctatatcaaatatgaagtctctggtaagacctactacgataacaacaactccgcaaactaccaagttagcacatcaaagccaaccacaacaactgctactgcgacaactacaaccgcaccaagcacttctactacaacacctcctagttcatctgagccagcaactttcccaactggtaattccactatttcttcttggatcaaaaaacaagagggtatctcaagattcgccatgcttagaaatatcaatcctccaggctctgcaacaggattcattgcagcatctttatcaactgcggggccagactactactacgcctggactagagatgcagctttgacatcaaatgtgattgtttatgaatacaacacaactttgtccggtaacaagacaatcttgaacgtcttgaaggattatgtgacattctctgtcaagactcaatctacatcaacagtttgtaactgtctcggcgaaccaaagttcaaccctgatggtagtggttacactggtgcttggggtagaccacaaaacgatggtccagcagagagagctacaactttcatcttgtttgctgactcttacctaacacaaaccaaggatgcaagctacgttactggaacactaaagcctgcaatctttaaagacctggactatgttgtaaacgtttggtcaaatggctgcttcgatctatgggaggaagtgaacggtgttcacttctacacattaatggtcatgagaaagggactcttgcttggtgcagactttgctaagagaaacggtgattctacacgtgcctccacttactcctccacagcttcaaccattgccaacaaaatctcttctttctgggtcagctcaaataactggattcaagtttctcaatcagttactggtggtgtttctaaaaagggcctggatgtgtcaaccttgcttgctgccaatttgggcagtgttgatgacgggttcttcaccccaggttctgaaaagatcctcgccaccgcagttgccgttgaagattcatttgctagtttatacccaatcaacaaaaatctaccatcataccttggaaattcaatcggtagatatccagaggatacatacaacggtaatggaaactctcagggtaacccttggtttcttgcagttacagggtacgctgaactgtactacagagcgattaaggaatggattggtaatggcggcgtaactgttagttctatttctctacctttcttcaaaaagttcgatagttctgcaacatctggtaaaaagtacacagtcggcacttccgattttaacaatttagctcagaacatagcactggcagctgatcgtttcttgagtacagtccaattgcatgcccataacaacggtagtttggctgaagagtttgatagaaccaccggtttatcaaccggcgccagagatttaacatggtcccatgcgtctttgataactgcttcttacgccaaggctggggcaccagctgcctga

SEQ ID NO: 7 - DNA, 1815 bp, Rhizopus delemar; identical to SEQ ID NO: 6
  source 1..1815: mol_type = genomic DNA

SEQ ID NO: 8 - DNA, 1818 bp, Rhizopus microsporus
  source 1..1818: mol_type = genomic DNA
atgaagctgatgaatcctagcatgaaagcatatgtgtttttcatcctctcatacttcagcttgctagttagttcggccgcagtacccacgtcggccgcggtccaagtggagtcgtataattatgacggaactaccttctcagggcgtatattcgtcaagaatattgcgtattccaaagtcgtcacagtaatctattcagatggctccgataattggaataataataacaacaaggttagcgccgcctattccgaggctatttctggatcaaactacgaatactggaccttctcggcgaagctgtcagggatcaaacagttttacgtcaagtacgaggtcagtggttcaacttactacgataataacggaaccaaaaattatcaggtccaggcgacgagcgcaacgtccacaactgcgacagccactaccactactgctaccgggactacgacaacctcgacaggaccgacgtccaccgcctctgtatcctttcccaccggaaacagcacaatttcgagctggataaaaaaccaagaggaaatctctcgcttcgctatgttacgtaacatcaatccccccggttcggcaactgggtttattgccgcatcattatctacagccgggcccgattactattatagctggactcgcgacagtgcactcacggctaatgtcatcgcatatgaatacaacacgactttcaccggcaatacgacccttcttaagtatttgaaagattatgtaactttctcagttaaaagtcaatcggttagtacggtctgtaattgtctcggtgaaccgaagtttaacgctgacgggtcctcgttcactggcccttgggggcgacctcagaacgacgggcccgcggaacgcgccgttacgttcatgctcattgcagactcatatctcacccagactaaagacgcgtcttatgtcactgggactttaaaaccagctatatttaaagatctggattacgttgtttctgtttggtcaaatgggtgttatgacttatgggaagaagtgaacggcgttcatttctacactttaatggtcatgcggaagggcctcattttaggggcggacttcgccgcacgtaatggagattcatcgcgcgcgtcaacatataaacaaacggcatcaactatggaaagtaaaatttctagcttctggtcggacagtaacaactacgttcaagtgtctcaatcggtaactgcgggggtaagcaagaagggacttgacgtgagtacactgcttgccgccaatattgggagcctaccagacgggttttttacacccggctcggaaaagattttagcaacggctgttgctcttgaaaacgcttttgcctcgctgtatccaatcaattcaaatttaccatcttatctgggaaatagtattggaaggtaccccgaggacacctataatgggaacggtaattcccaaggtaacccttggttcttggctgtgaatgcctatgccgagttgtactatcgcgcaattaaggaatggataagtaatggcaaagtgacggtttcaaacatctccctaccttttttcaaaaaattcgactccagtgcgacttctggaaaaacctatacagcgggcacctccgacttcaataatctcgcgcagaatattgcactcggagcagaccgatttctttctacagtgaaattccatgcgtacacgaacggtagcttgtcagaagagtacgaccggtctaccggcatgtcaacgggagcacgagatcttacttggtcccatgcaagtttaattactgtggcatacgctaaagcagggtcgccagcggcataa

SEQ ID NO: 9 - DNA, 1800 bp, synthetic construct
  misc_feature 1..1800: note = Mfa2-Rhizopus oryzae
  source 1..1800: mol_type = other DNA
atgaaattcatttctacctttctcacttttattttagcggccgtttctgtcactgctggtgcctcgatccccagctcggccagcgtccaactggactcgtataattatgacggatctaccttctcagggaaaatatacgtcaagaatattgcgtattccaaaaaagtcacagtagtctatgccgatggctccgataattggaataataatggaaacacaattgcggcctcattttccgggcctatttctggatcaaactacgaatactggaccttctcggcgtcggtgaaagggatcaaagagttttacattaagtacgaggtcagtggtaaaacttactacgataataacaactcagctaattatcaggtcagcacgagcaagccgactacaactacggcagccactaccactactactgccccgtctacgagtaccacaacacggccgagttcctcagaacctgcaacttttcccaccggaaacagcacaatttcgagctggataaaaaagcaagaggatatctctcgcttcgctatgttacgtaacatcaatccccccggttcggcaactgggtttattgccgcatcattatctacagccgggcccgattactattatgcgtggactcgcgacgcggcactcacgtctaatgtcatcgtatatgaatacaacacgactctatcaggcaataagaccatccttaacgttttgaaagattatgtaactttctcagttaaaacgcaatcgacttcgaccgtctgtaattgcttgggcgagccaaaattcaatccggacggttcgggatataccggtgcttggggccgtccgcagaacgacggcccggccgaacgagctacgacgttcgtattattcgcggattcatacttgacgcaaactaaggacgcttcctatgttacgggtactttaaagcctgcaatttttaaagaccttgactatgttgttaatgtctggtcaaacggttgtttcgatttgtgggaagaggtgaatggtgttcacttctatactctgatggttatgcggaaaggattattactaggggcagactttgcaaaacgaaacggtgattcgaccagagcctcgacttattctagcacagcctccacgatcgcaaataaaattagcagtttctgggtaagtagtaacaactgggtccaggtttctcagtcggttacgggcggcgtaagtaagaaggggcttgatgtctcaaccctactggcggcaaacctgggttccgtagatgatggatttttcactcctggaagcgaaaaaattcttgccacagctgttgccgtagaggattcgtttgcttcattatatccaattaataagaacttaccgtcttacctgggaaatgcaataggccgatatccggaggatacctataatggtaacggtaatagccaaggtaacccttggtttcttgcggtcacaggttatgcagaactgtattacagagcgatcaaagaatggatatctaatggaggagttacagtttcatcgatttctctccctttcttcaaaaagtttgactcctcagctacaagtggcaaaaaatacacggtcggtacaagcgactttaataacctcgcacagaacatcgcccttgctgccgataggttcctgagcactgtgcaacttcatgcaccgaacaacggttcattggcagaagagttcgaccgaactaccggtttctccactggagcgcgtgatttaacgtggagtcatgcttcgctgatcacagcgtcgtatgctaaggcaggcgccccggctgcctaa

SEQ ID NO: 10 - DNA, 1548 bp, Saccharomycopsis fibuligera
  source 1..1548: mol_type = genomic DNA
atgataaggctcactgttttcctcaccgcagtcttcgctgcggtcgcatcatgcgtgccggtcgagttggacaagcgaaacacaggccacttccaagcgtattctgggtacacagttgcccgttcgaactttacccagtggatacatgagcagcccgcagtttcttggtattatttacttcaaaacatcgattatcccgaaggccaatttaaatctgctaaacctggagtagtagttgcgtcaccctcaaccagtgaacccgattacttttaccagtggacgagagatacagcaataacattccttagtcttattgcagaagtggaagaccacagtttttcgaacactaccttagcgaaggttgttgagtactatatttccaatacatatacactacagagggtaagcaatccatctgggaactttgattcacctaatcatgatgggttaggggagcccaagttcaacgtggacgataccgcctatacagcttcatggggccggccacagaacgatggaccggcactacgtgcgtatgcgatttcgcgttatctcaatgccgttgctaagcataataatggcaaactcctattagcgggccaaaatggaatcccttatagttcagcgtcagatatatattggaagatcattaaaccggacctacagcacgtttctacccactggtccacttcggggttcgatctatgggaagaaaaccaaggcacccacttttttactgccttagtacaactaaaagctcttagttatggaatccctctctccaaaacgtacaatgaccctgggttcacttcgtggttggaaaaacaaaaggatgctctaaacagctacattaactcatccggctttgtgaactcgggaaaaaagcacatcgtcgagtccccgcaattaagtagccgtggtggcttagactctgctacttacattgcagctttgattacgcatgacattggtgatgatgatacctatacgccttttaacgttgataattcatacgtgcttaattctctatactatttactggtcgataacaagaatcggtataaaataaacggaaactataaggctggcgcagctgtcggacgctaccccgaggatgtctataacggagtcggtacgtcagagggcaatccttggcagctagcaacagcgtacgcaggacaaaccttctatactctcgcatataacagtctaaagaacaagaagaatctcgtgatagagaagcttaattatgatttgtacaacagtttcatagcggatttgtcgaaaatcgactcctcgtatgcttcgaaggattctttaacccttacatatggttcagacaactataagaatgttatcaaatctctattacaattcggagatagttttctcaaggtattgctagaccatatcgatgacaacggtcaattgaccgaagagattaataggtatactgggtttcaagctggcgcggtcagtttgacgtggagtagtgggtcattgttaagtgcgaatcgagcacggaataagttaatcgagttattataa

SEQ ID NO: 11 - DNA, 1920 bp, Aspergillus kawachii
  source 1..1920: mol_type = genomic DNA
atgagcttccggtccttgctggcattgagtggcctagtttgctcaggacttgcgagtgtgattagtaaaagagcaaccctcgactcctggctctccaacgaagctacggtagcacgtaccgctatcctaaataatatcggcgcggatggagcgtgggtatctggtgcggattccggtatcgtcgtagcatcaccttcaactgataatcccgattatttttatacttggacacgggatagcggccttgtcattaagactttggttgaccttttcagaaatggggacaccgacctcctgtcgacgatcgagcattatatatcaagccaagcgataatacaaggagtatctaatcctagcggggatttgtcgagtggcggtttgggcgagcccaagttcaacgtggacgagactgcatatacgggatcatggggccgtcctcaacgagatggaccagcgctacgcgccaccgctatgattggctttggccagtggctgctagataacgggtacacatctgcggctacggaaatcgtttggccattggtccgtaatgacctttcatatgtcgctcagtactggaaccaaactggctacgatttatgggaggaagtgaatggtagctcatttttcaccattgccgtgcagcaccgggcgttagttgaaggatcggcctttgcaacggcggttggatcatcctgtagctggtgtgatagccaagcccctcaaattctatgttaccttcaatcattctggacaggtagttacatccttgctaatttcgattccagtcggtccgggaaagacacgaatacactcttgggctccattcacacctttgacccggaggcgggctgcgatgattcaactttccagccatgctctccaagagcccttgcaaatcacaaagaagtggtggattcctttcgtagcatttatactctcaatgacggtttgtccgactcagaggctgttgctgttggccgatatccggaagatagctattataatggcaacccgtggtttttatgcacattagctgcggccgaacagctctatgacgctttataccagtgggacaaacagggttcactagaaatcacagatgtgtcactcgattttttcaaggccttgtactcaggagccgctactgggacatactcgtcgagtagttcgacatattcaagcattgtttcggcagttaagacgttcgcggacgggttcgtcagcatagtagagacacatgccgccagtaacgggtcgctaagcgaacaattcgataaatcggatggagatgaactcagcgctcgtgatcttacctggtcttatgccgcactgttaacagccaataatcgtcgtaactctgttgtgccacctagttggggagagacatccgcaagctcagtccccgggacgtgtgccgccacctccgcatccggtacgtattccagtgttaccgttaccagctggccatctattgtagctacgggtggaacaacgaccaccgctacgacgactggcagtggaggtgtaacttcaacatctaaaacaacgaccacagcgtctaagacttctaccactacaagttcaacctcctgcacgacccctacagcggtggccgttacattcgacctcacggccaccaccacttacggggaaaacatttacctagtggggtctatatcccaattaggagactgggagacttcagatggaatcgcgctatcggccgataaatatacgtcctctaacccgttatggtatgtgacagtaactttaccagcgggagagagcttcgaatataagttcatccgagtggaatcagatgatagcgtggagtgggagtcggacccaaatcgggagtatactgtccctcaggcttgcggtgagtccactgctaccgtaacggatacatggcgctaa

SEQ ID NO: 12 - DNA, 1911 bp, Aspergillus terreus
  source 1..1911: mol_type = genomic DNA
atgacgaggatcttgactctggcattgcacggcctagctctggtccagtcagtggtgggggccccgcaactagcaccccgggcaaccacgtcgttggacgcctggctggcatcggaaaccactgtagcattagatggaatcctggataacgtgggctcgtctggtgcgtatgctaaatcagccaagtcgggcattgtcattgcctccccctccacttccgatcctgactactactatacgtggacccgagatgcggctttgactgtaaaagcactaatcgacctatttcggaacggggagacatcattgcagaccgtgattatggagtacatctcgtcgcaagcctatctgcaaactgtaagtaatccttccggctcgctttcgacgggcggtctggcagaacctaaatattatgttgatgagactgcgtacaccggaagttgggggcggcctcaacgagatggaccagcgctacgcgcaacggcaatgattgactttgggaattggttaattgacaatggctattctacatatgcctcatccattgtatggcctatagtccgtaatgacctttcttatgtagcccagtattggaaccaaactgggtatgatttgtgggaggaggtaaacggttcttcattcttcaccattgcagtgcagcatagagccttggtcgagggctcaaccttcgcttccaaagtcggtgcatcttgctcatggtgtgactctcaggctccacaggtcctttgttttctccaacgcttctggactgggtcttacataatggcaaactttggcggtggtaggtcaggtaaggacgcgaacaccgtgcttggttcaattcacacgttcgaccctaacgcgggctgtgacgatacgacttttcagccgtgttccccccgtgcgttagctaatcacaaagtatataccgatagctttcggtccatttattccattaattcagggatttccagcggtaaagctgtcgcggtgggccgctatccggaggattcttactataatggaaacccctggtttttaacgacgctcgcggctgccgagcaactatatgacgctatctatcagtggcaaaaaataggcagtattactattacggacgtgtcgctcgcgttcttcaaggatctttactcttctgcggcggtagggacatatgcaagtagtagtagcgcctttacctcaattgtgagcgcggtaaagacgtatgctgacggctatatgtccatcgttcaaacacacgctatgactaatggctcgttatccgaacagttcggtaagtcagatggcttttctctatctgctagggacttaacgtggtcgtacgcagccctactgaccgccaatctgaggcgtaattccgtcgttccaccttcctggggtgaaacgactgccacttcagtgccctcggtttgttcggctacgtctgcaacagggacctattctacggcgactaatacagcatggccatctaccctcacttctggaacgggcgcaacgactacgacttctaaagctacaagttcatcaactacgacgacctcttcggcgagctcaactacagtagagtgcgtggtccccaccgctgtagcggtcacatttgacgaggtggcgactacgacttatggtgagaacgtatacgttgtcggcagtatcagtcagctcggctcttgggatacgtccaaagcagtggctttatctgcgtcgaagtatacttcgagcaacaacctgtggtatgttacggtaacccttccggctggcaccactttccagtacaagttcatccgggtatcatcgtcgggttccgtcacttgggaaagcgatccgaatcgctcttatacagtgccctcggcctgtggtacgtcaacagctgtcgtcaataccacttggcgctaa

SEQ ID NO: 13 - DNA, 1854 bp, Thermomyces lanuginosus
  source 1..1854: mol_type = genomic DNA
atgctgttccagcctactctgtgcgccgcacttgggttagcggccctcatcgtgcagggcggcgaggcacgcccggagactactgtgccacacgctaccggttcgctagatgatttccttgcggctcagagccccatcgcttttcagggcattttaaataatataggaccctccggcgcttattccgaaggtgttaatcccggtgtagtaatcgctagcccctcaaaacaagaccctgattatttctatacatgggtcagggacgccgcactcacggtacagtatctagtcgaagagttggtggcgggaaatgcatcgttacaatttctgattcaagactacatctcttcccaagcacgactccagacggtggagaacccttcgggtagcctatcatccggcggtttaggtgaaccgaaattccacgtcgacgagacagcgttcactgattcctggggacgcccccaacgagatgggccaccattaagggctatagctatgatttccttcgctaattatttaatagataatggccatcaatcgacagttgaggatattatctggcccattgttagaaatgacctttcttacgtcagccaacattggaacgagacaacattcgatatttgggaggaggtccattcgagtagctttttcaccaccgccgtgcaatatcgagctttggttcaaggtagtgctctagcctctaaactaggtcacacttgcgacaattgtggttctcaggctccccagatcttgtgctttctacagtcctactggactggctcccatatacttgctaacacgggtggcggtaggagcggaaaggatgtaagtaccatcctcggcgtgattggtagtttcgatcctaatgctgactgtgatgatgtaactttccaaccctgtagcgcccgggctttagctaatcataaacaagtggttgatagctttcgctctatctacgcgatcaatgctgggatcccttctgggtcagctgtagcagtcggacgttatccggaggacgtgtatcagggtggccacccttggtacttgacgaccgcagctgccgctgagcagctttatgacgccatatatcaatggaaccacgtgggacacatagacatcaacgctgtcaacttagatttcttcaaaagcatatacccgagtgcggcagaaggaacgtacacaagcgattcatcaacctttcaggacataatcagtgcggttcgcacatatgccgacggtttcttgtctgtaatagaaaaatataccccaccggataaccttttagccgaacaattccatcgtgagacaggtatacctctcagcgcagccagtctgacctggtcatacgcggctttgaataccgctgcacaacgcagggcttccatagttccctccccctggaatagtaatagcactgacctaccggataaatgtagtgcgacttcagcaacaggtccatatgccacacctactaacacggcctggccgactacgactcagcctcccgaacggccggcctgtactccgccgtcagaagtaacgctgacctttaacgcactcgtagacaccgcctttggtcagaacatctacttggtgggaagcatacctgagttgggctcttgggacccagcaaatgccttgctaatgagtgcaaagtcatggacctctgggaatcctgtatggactttatctatatcgctacctgctggaacgtcgttcgagtacaaatttatacgcaaagacgatggctcatctgacgtggtatgggagtcggacccaaatcggtcgtataatgtccctaaggattgcggtgcgaatactgctaccgtaaactcctggtggcgctaa

SEQ ID NO: 14 - DNA, 2045 bp, synthetic construct
  misc_feature 1..2045: note = Mfa2-Neurospora crassa
  source 1..2045: mol_type = other DNA
atgaaattcatttctacctttctcacttttattttagcggccgtttctgtcactgctgacgcgatctataatctgaagcaagtacttctatctaaccatgactttacgacgagcttggtgtccaacgcaaccgacttctccacgtcgcccctgacctatttcgcaatgcatttggtttcgagtttacttgtagtcggggctgcattccaagcagttttagggttgcctgatccccttcacgagaaacgccattctgatattatcaaacgttccgtcgattcgtacatccaaacggaaacccccattgcgcaaaagaacctactttgcaacatcggagcaagcggatgccgagcctccggagccgcgtccggggtggtagtcgcatcgccttcaaaaagcagtcctgattactggtatacttggacccgggatgcagcgctagtgacaaagttgatcgttgacgagtttactaatgattataataccacgttacagaacaccatccaggcatacgcggctgcccaagctaagttgcaaggcgtcagtaacccatccggaagcctcagtaatggggctgggttaggagaacccaagtttatggttgatctacaacaatttaccggtgcatggggtaggccccaacgagatgggccccctctgcgtgcgatcgctttgatagggtacggaaagtggttagtctcgaacggctatgcagacacggctaagtcaattatttggcccatcgtcaagaatgatttagcctatacagctcagtattggaataacactggatttgacctatgggaagaagttaactcctccagtttctttacgattgcggcgtcccaccgggctttggttgaagggtcagctttcgcgaagtccgtgggctcctcatgtagcgcgtgcgacgctatagcgccccaaatcttgtgctttcaacagagcttttggtcaaatagcggttatattatctccaactttgtcaattaccgatcgggtaaagatattaattcagtcctaacttccatacataattttgatccggcggccggttgtgacgtaaatactttccaaccttgctcggatcgggctttagcgaaccacaaggtcgtagttgatagtatgcgattctggggtgtgaactcaggtaggaccgcaggcaaagctgcggcagtgggacggtacgcggaggacgtttattacaatggtaacccatggtacctagcaacgctagcggcagccgagcagctatacgacgccgtctatgtctggaagaagcagggaagtataactgttacatccacctcgttggcattttttaaggacttagttccttcagtctcgactggtacctacagctctagttcttctacatatactgcgatcattaacgctgtaacgacatatgcagacggctttgtcgacatagttgcccaatatactccatccgatgggtccttggcggaacaatttgataaggattcgggtgccccattgagcgctacacacctaacctggtcttacgcgtcttttctatcggctgctgcaaggcgcgcagggattgtgcctccatcctggggtgcagcgtcagccaatagtctgcccggttcgtgcagcgcctctacagtagcaggaagttatgccaccgctacagcgacctcgtttccggcaaacctgactccggcttcaactacagtgacaccacctacccaaacaggctgcgcagcagatcatgaagttctggttactttcaacgaaaaagttacgacaagttatggtcagacggtaaaggtggtaggttctatagcagcccttgggaattgggcccctgcgagcggagtgacgctctcggcaaaacagtactcctcctcaaatccattatggtctacgaccattgctttgcctcaagggacctcgtttaaatataaatatgttgtcgttaatagtgatggatctgtaaaatgggagaatgatcccgatcgcagctatgccgtaggaacagattgtgcttccacagccactcttgatgatacttggaggta

SEQ ID NO: 15 - DNA, 4863 bp, synthetic construct
  misc_feature 1..4863: note = Mfa2-Rhizopus oryzae GA integration construct
  source 1..4863: mol_type = other DNA
ctaaattcggccttgctcagagactcctggattttggctaacaacgcagtcccttcgatgcatatagctaggccacaaattatgccaataacggtccatgggttgatgttttcttgaattctttcgtttttcatgctatttgcgtcttcccaagtcccagcgttccagtattcatactgcgcgttagagtggtagccataagagccggcatattggtaattttcagtattaacgttagaacgtggtgaatacgatgtggtccagccttgcctcgttgtgtcatatacgatctttttctttgggtcacaaagaatatcatatgcttgagagatgactttaaatctatgtagtttttcgcttgatgttagcagcagcggtgatttactatcactgttggtaaccttttctgagctaaatatttgaatgttatcggaatggtcagggtggtacaattttacataacgatgatattttttttttaacgacttcttgtccagtttaggatttccagatccggcctttggaatgccaaaaatatcatagggagttggatctgccaactcaggccattgttcatcccttatcgtaagttttctattgccatttttatcgttcgctgtagcatacttagctataaaagtgatttgtgggggacacttttctacacatgataagtgccacttgaataaaaatgggtatacgaacttatggtgtagcataacaaatatattgcaagtagtgacctatggtgtgtagatatacgtacagttagttacgagcctaaagacacaacgtgtttgttaattatactgtcgctgtaatatcttctcttccattatcaccggtcattccttgcaggggcggtagtacccggagaccctgaacttttctttttttttttgcgaaattaaaaagttcattttcaattcgacaatgagatctacaagccattgttttatgttgatgagagccagcttaaagagttctcgagatctcccgagtttatcattatcaatactgccatttcaaagaatacgtaaataattaatagtagtgattttcctaactttatttagtcaaaaaattggccttttaattctgctgtaacccgtacatgcccaaaatagggggcgggttacacagaatatataacatcataggtgtctgggtgaacagtttattcctggcatccactaaatataatggagcccgctttttttaagctggcatccagaaaaaaaaagaatcccagcaccaaaatattgttttcttcaccaaccatcagttcataggtccattctcttagcgcaactacacagaacaggggcacaaacaggcaaaaaacgggcacaacctcaatggagtgatgcaacctgcttggagtaaatgatgacacaaggcaattgacctacgcatgtatctatctcattttcttacaccttctattaccttctgctctctctgatttggaaaaagctgaaaaaaaaggttgaaaccagttccctgaaattattcccctatttgactaataagtatataaagacggtaggtattgattgtaattctgtaaatctatttcttaaacttcttaaattctacttttatagttagtcttttttttagtttaaaacaccaagaacttagtttcgaataaacacacataaacaaacaaatctagaatgaagttcatttccactttcttgaccttcattttggctgctgtctctgtcaccgctgcatctattccatctagtgcatctgtacaattggactcctacaattacgatggttccacattttccggcaagatttatgtcaaaaacatcgcttactctaaaaaggttactgttgtgtacgcagacggttctgacaactggaacaataacggcaacactattgctgcatcattttcaggcccaatctctggatcaaattacgaatactggacattctcagcatcagtgaagggcataaaggagttctacatcaaatacgaagtttcaggtaagacatattacgacaataacaactctgcaaactaccaagtctcaacttctaaacctactacaactactgcagctacaaccacaactacagctccatcaacttctacaacaacccgtccatctagttcagagcctgccaccttccctactggtaattctaccatcagctcttggatcaaaaagcaggaagatatttccagattcgctatgcttagaaacatcaacccacctggttctgccacagggtttatcgccgcatcactctctaccgctggtccagattactactacgcgtggacaagagatgccgctttgacatctaacgttatcgtttacgaatacaacaccacattgtctgggaataagacaattctaaacgtacttaaggattacgtcacattcagtgttaagacacagtctacttcaacagtttgtaattgccttggtgaaccaaagttcaatccagacggcagtggttacacaggtgcttggggtagacctcaaaatgatggtcctgcagaaagagcgactacatttgttctgtttgccgacagctacttgactcaaactaaggatgcctcatacgtcactggtacattaaagccagcaattttcaaagatctcgattacgttgttaacgtctggagtaacggatgtttcgatttatgggaggaggtgaacggagttcatttctacacccttatggttatgagaaaagggctattgttgggggctgatttcgcgaagagaaacggtgactcaactagagcctcaacttactcttctactgcttccacaattgctaacaagatatcaagtttctgggttagctcaaacaactgggtgcaagtatcccaatctgtcacaggaggtgtaagtaaaaaggggttagacgttagcaccctgttagctgcgaatctaggatcagtcgatgatggatttttcactccaggttctgaaaagatattagctacagctgtggcagtcgaagattcctttgccagtctatacccaatcaacaaaaaccttccatcatacttggggaacgctattggaagataccctgaagatacatacaacggtaatggtaactcacaaggcaatccttggtttctggcggttaccggctacgcagagttgtactatagagcaattaaggaatggatttctaatggaggcgttacagtgtcctctatctcattgccatttttcaaaaagttcgatagctctgcaacatccggtaaaaagtacaccgtaggtacttctgacttcaacaatttagcacaaaacattgctcttgctgcagatcgtttcctatctactgtacaactccatgcaccaaacaatggttcattagcagaggaatttgatagaacaacaggtttttctaccggcgctagagatttaacatggtcccacgcctcattgataacagcatcctatgccaaagccggtgctccagctgcataattaattaaacaggccccttttcctttgtcgatatcatgtaattagttatgtcacgcttacattcacgccctcctcccacatccgctctaaccgaaaaggaaggagttagacaacctgaagtctaggtccctatttatttttttatagttatgttagtattaagaacgttatttatatttcaaatttttcttttttttctgtacaaacgcgtgtacgcatgtaacgggcagacggccggccataacttcgtataatgtatgctatacgaagttatggcaacggttcatcatctcatggatctgcacatgaacaaacaccagagtcaaacgacgttgaaattgaggctactgcgccaattgatgacaatacagacgatgataacaaaccgaagttatctgatgtagaaaaggattagagatgctaagagatagtgatgatatttcataaataatgtaattctatatatgttaattaccttttttgcgaggcatatttatggtgaaggataagttttgaccatcaaagaaggttaatgtggctgtggtttcagggtccataaagcttttcaattcatcttttttttttttgttcttttttttgattccggtttctttgaaatttttttgattcggtaatctccgagcagaaggaagaacgaaggaaggagcacagacttagattggtatatatacgcatatgtggtgttgaagaaacatgaaattgcccagtattcttaacccaactgcacagaacaaaaacctgcaggaaacgaagataaatcatgtcgaaagctacatataaggaacgtgctgctactcatcctagtcctgttgctgccaagctatttaatatcatgcacgaaaagcaaacaaacttgtgtgcttcattggatgttcgtaccaccaaggaattactggagttagttgaagcattaggtcccaaaatttgtttactaaaaacacatgtggatatcttgactgatttttccatggagggcacagttaagccgctaaaggcattatccgccaagtacaattttttactcttcgaagacagaaaatttgctgacattggtaatacagtcaaattgcagtactctgcgggtgtatacagaatagcagaatgggcagacattacgaatgcacacggtgtggtgggcccaggtattgttagcggtttgaagcaggcggcggaagaagtaacaaaggaacctagaggccttttgatgttagcagaattgtcatgcaagggctccctagctactggagaatatactaagggtactgttgacattgcgaagagcgacaaagattttgttatcggctttattgctcaaagagacatgggtggaagagatgaaggttacgattggttgattatgacacgc

SEQ ID NO: 16 - DNA, 4748 bp, synthetic construct
  misc_feature 1..4748: note = Mfa2-Rhizopus oryzae GA integration construct
  source 1..4748: mol_type = other DNA
ggccgctccatggagggcacagttaagccgctaaaggcattatccgccaagtacaattttttactcttcgaagacagaaaatttgctgacattggtaatacagtcaaattgcagtactctgcgggtgtatacagaatagcagaatgggcagacattacgaatgcacacggtgtggtgggcccaggtattgttagcggtttgaagcaggcggcggaagaagtaacaaaggaacctagaggccttttgatgttagcagaattgtcatgcaagggctccctagctactggagaatatactaagggtactgttgacattgcgaagagcgacaaagattttgttatcggctttattgctcaaagagacatgggtggaagagatgaaggttacgattggttgattatgacacccggtgtgggtttagatgacaagggagacgcattgggtcaacagtatagaaccgtggatgatgtggtctctacaggatctgacattattattgttggaagaggactatttgcaaagggaagggatgctaaggtagagggtgaacgttacagaaaagcaggctgggaagcatatttgagaagatgcggccagcaaaactaaaaaactgtattataagtaaatgcatgtatactaaactcacaaattagagcttcaatttaattatatcagttattacccgggaatctcggtcgtaatgatttttataatgacgaaaaaaaaaaaattggaaagaaaaagcttcatggcctttataaaaaggaaccatccaatacctcgccagaaccaagtaacagtattttacggggcacaaatcaagaacaataagacaggactgtaaagatggacgcattgaactccaaagaacaacaagagttccaaaaagtagtggaacaaaagcaaatgaaggatttcatgcgtttgataacttcgtataatgtatgctatacgaagttatctcgagggccagaaaaaggaagtgtttccctccttcttgaattgatgttaccctcataaagcacgtggcctcttatcgagaaagaaattaccgtcgctcgtgatttgtttgcaaaaagaacaaaactgaaaaaacccagacacgctcgacttcctgtcttcctgttgattgcagcttccaatttcgtcacacaacaaggtcctagcgacggctcacaggttttgtaacaagcaatcgaaggttctggaatggcgggaaagggtttagtaccacatgctatgatgcccactgtgatctccagagcaaagttcgttcgatcgtactgttactctctctctttcaaacagaattgtccgaatcgtgtgacaacaacagcctgttctcacacactcttttcttctaaccaagggggtggtttagtttagtagaacctcgtgaaacttacatttacatatatataaacttgcataaattggtcaatgcaagaaatacatatttggtcttttctaattcgtagtttttcaagttcttagatgctttctttttctcttttttacagatcatcaaggaagtaattatctactttttacaagtctagaatgaagtttatctccacgtttttaacctttatcctagcagctgtcagcgtcaccgccgcatcaattccgagttcagcatctgtacaacttgactcttacaattacgatggcagcactttctcagggaaaatttatgtgaaaaacatagcatatagtaagaaggttaccgtggtatatgcagacggttctgataattggaataataatggaaacactattgccgccagtttttccggcccaatttctggttccaattacgagtattggaccttttctgcatcagtaaaaggcatcaaggaattctatattaagtacgaagtttcaggtaagacatattacgataacaataactcagcaaattatcaagtctctacatctaagcccacaacaacaactgctgctaccaccactacaaccgctccttctaccagcaccactaccagaccaagctctagtgaaccggctacctttcctaccggaaacagtaccatctcaagctggatcaaaaagcaagaggacataagtcgttttgctatgttgaggaacattaatcctccaggatccgcgaccggtttcattgcagcatcactaagtactgccgggcctgattattattatgcttggactagagacgctgcattaacatcaaacgtgattgtttatgaatataatacgaccctttccggtaataaaacgatcttgaacgtattaaaagactatgtgacctttagtgtgaagacccaatctacatctacagtgtgtaattgtttgggagaacctaaattcaatccagacggttctgggtacactggtgcctggggtagacctcaaaacgacggtccagcagaaagagcaacaacctttgttctatttgctgactcttatttaacgcaaacaaaggacgcctcatatgttacagggaccctaaaaccagcaattttcaaagacttggattatgttgttaatgtttggagcaacggatgttttgacttgtgggaggaggttaacggtgtacacttttatacattgatggtgatgagaaaagggttgctattgggagcagatttcgctaaaagaaatggtgattctacaagagcgagcacatatagtagcaccgcttcaacaatcgccaataaaatctcatctttctgggtatctagcaacaactgggtacaagtttcccaaagtgttaccggcggtgtgtccaaaaagggtttagacgttagcacacttctagctgctaatttgggtagcgttgatgacgggttttttactccaggtagtgagaagatactggcaaccgcggtggcggttgaagacagctttgcttcattgtatcctataaataaaaatctgccctcttatctgggtaatgcaattggcagatacccagaagatacctacaatggtaatggtaattcccaggggaacccatggtttttggctgttacaggctacgcagaactttattaccgtgcaatcaaggaatggatttcaaatggcggcgtcactgtcagtagtataagtttgcccttttttaagaaatttgattcctcagcaacgtctggtaaaaaatacaccgtaggtactagtgatttcaataatttggcccaaaatattgcgcttgctgctgacaggtttcttagtaccgttcagttgcacgctccaaataatggctcattggctgaagaatttgatcgtacgacaggtttctccactggtgctagggatttgacttggagtcatgcctccttaatcacagcaagctatgctaaagctggtgcacctgctgcttagttaattaatttaccagcttactatccttcttgaaaatatgcactctatatcttttagttcttaattgcaacacatagatttgctgtataacgaattttatgctatttttttaatttggagttcggtgatgaaagtgtcacagcgaatttcctcacatgtagggaccgaattgtttacaagttctctgtaccaccatggagacatcaaagattgaaaatctatggaaagatatggacggtagcaacaagaatatagcacgagccgcggagttcatttcgttacttttgatatcgctcacaactattgcgaagcgcttcagtgaaaaaatcataaggaaaagttgtaaatattattggtagtattcgtttggtaaagtagagggggtaatttttcccctttattttgttcatacattcttaaattgctttgcctctccttttggaaagctatacttcggagcactgttgagcgaaggctcaggccggcagcacgcagcacgctgtatttacgtatttaattttatatatttgtgcatacactactagggaagacttgaaaaaaacctaggaaatgaaaaaacgacacaggaagtcccgtatttactattttttccttccttttgatggggcagggcggaaatagaggataggataagcctactgcttagctgtttccgtctctacttcggtagttgtctcaattgtcgtttcagtattacctttagagccgctagacgatggttgagctatttgttgagggaaaactaagttcatgtaacacacgcataacccgattaaactcatgaatagcttgattgcaggaggctggtccattggagatggtgccttattttccttataggcaacgatgatgtcttcgtcggtgttcaggtagtagtgtacactctgaatcagggagaaccaggcaatgaacttgttcctcaagaaaatagcggccataggcatggattggttaaccacaccagatatgcttggtgtggcagaatatagtccttttggtggcgcaattttcttgtacctgtggtagaaagggagcggttgaactgttagtatatattggcaatatcagcaaatttgaaagaaaattgtcggtgaaaaacatacgaaacacaaaggtcgggccttgcaacgttattcaaagtcattgtttagttgaggaggtagcagcggagtatatgtattccttttttttgcctatggatgttgtaccatgcccattctgctcaagcttttgttaaaattatttttcagtattttttcttccatgttgcgcgttacgagaacagaagcgacagataaccgcaatcatacaactagcgctactgcggggtgtaaaaagcacaagaactaagccaagatcacaacagttat

SEQ ID NO: 17 - DNA, 1674 bp, synthetic construct
  misc_feature 1..1674: note = Integration construct
  source 1..1674: mol_type = other DNA
ctaaattcggccttgctcagagactcctggattttggctaacaacgcagtcccttcgatgcatatagctaggccacaaattatgccaataacggtccatgggttgatgttttcttgaattctttcgtttttcatgctatttgcgtcttcccaagtcccagcgttccagtattcatactgcgcgttagagtggtagccataagagccggcatattggtaattttcagtattaacgttagaacgtggtgaatacgatgtggtccagccttgcctcgttgtgtcatatacgatctttttctttgggtcacaaagaatatcatatgcttgagagatgactttaaatctatgtagtttttcgcttgatgttagcagcagcggtgatttactatcactgttggtaaccttttctgagctaaatatttgaatgttatcggaatggtcagggtggtacaattttacataacgatgatattttttttttaacgacttcttgtccagtttaggatttccagatccggcctttggaatgccaaaaatatcatagggagttggatctgccaactcaggccattgttcatcccttatcgtaagttttctattgccatttttatcgttcgctgtagcatacttagctataaaagtgatttgtgggggacacttttctacacatgataagtgccacttgaataaaaatgggtatacgaacttatggtgtagcataacaaatatattgcaagtagtgacctatggtgtgtagatatacgtacagttagttacgagcctaaagacacaacgtgtttgttaattatactgtcgctgtaatatcttctcttccattatcaccggtcattccttgcaggggcggtagtacccggagaccctgaacttttctttttttttttgcgaaattaaaaagttcattttcaattcgacaatgagatctacaagccattgttttatgttgatgagagccagcttaaagagttctcgagatctcccgagtttatcattatcaatactgccatttcaaagaatacgtaaataattaatagtagtgattttcctaactttatttagtcaaaaaattggccttttaattctgctgtaacccgtacatgcccaaaatagggggcgggttacacagaatatataacatcataggtgtctgggtgaacagtttattcctggcatccactaaatataatggagcccgctttttttaagctggcatccagaaaaaaaaagaatcccagcaccaaaatattgttttcttcaccaaccatcagttcataggtccattctcttagcgcaactacacagaacaggggcacaaacaggcaaaaaacgggcacaacctcaatggagtgatgcaacctgcttggagtaaatgatgacacaaggcaattgacctacgcatgtatctatctcattttcttacaccttctattaccttctgctctctctgatttggaaaaagctgaaaaaaaaggttgaaaccagttccctgaaattattcccctatttgactaataagtatataaagacggtaggtattgattgtaattctgtaaatctatttcttaaacttcttaaattctacttttatagttagtcttttttttagtttaaaacaccaagaacttagtttcgaataaacacacataaacaaacaaat

SEQ ID NO: 18 - DNA, 4260 bp, synthetic construct
  misc_feature 1..4260: note = Mfa2-Rhizopus oryzae integration construct
  source 1..4260: mol_type = other DNA
tcgagatctcccgagtttatcattatcaatactgccatttcaaagaatacgtaaataattaatagtagtgattttcctaactttatttagtcaaaaaattggccttttaattctgctgtaacccgtacatgcccaaaatagggggcgggttacacagaatatataacatcataggtgtctgggtgaacagtttattcctggcatccactaaatataatggagcccgctttttttaagctggcatccagaaaaaaaaagaatcccagcaccaaaatattgttttcttcaccaaccatcagttcataggtccattctcttagcgcaactacacagaacaggggcacaaacaggcaaaaaacgggcacaacctcaatggagtgatgcaacctgcttggagtaaatgatgacacaaggcaattgacctacgcatgtatctatctcattttcttacaccttctattaccttctgctctctctgatttggaaaaagctgaaaaaaaaggttgaaaccagttccctgaaattattcccctatttgactaataagtatataaagacggtaggtattgattgtaattctgtaaatctatttcttaaacttcttaaattctacttttatagttagtcttttttttagtttaaaacaccaagaacttagtttcgaataaacacacataaacaaacaaatctagaatgaagttcatttccactttcttgaccttcattttggctgctgtctctgtcaccgctgcatctattccatctagtgcatctgtacaattggactcctacaattacgatggttccacattttccggcaagatttatgtcaaaaacatcgcttactctaaaaaggttactgttgtgtacgcagacggttctgacaactggaacaataacggcaacactattgctgcatcattttcaggcccaatctctggatcaaattacgaatactggacattctcagcatcagtgaagggcataaaggagttctacatcaaatacgaagtttcaggtaagacatattacgacaataacaactctgcaaactaccaagtctcaacttctaaacctactacaactactgcagctacaaccacaactacagctccatcaacttctacaacaacccgtccatctagttcagagcctgccaccttccctactggtaattctaccatcagctcttggatcaaaaagcaggaagatatttccagattcgctatgcttagaaacatcaacccacctggttctgccacagggtttatcgccgcatcactctctaccgctggtccagattactactacgcgtggacaagagatgccgctttgacatctaacgttatcgtttacgaatacaacaccacattgtctgggaataagacaattctaaacgtacttaaggattacgtcacattcagtgttaagacacagtctacttcaacagtttgtaattgccttggtgaaccaaagttcaatccagacggcagtggttacacaggtgcttggggtagacctcaaaatgatggtcctgcagaaagagcgactacatttgttctgtttgccgacagctacttgactcaaactaaggatgcctcatacgtcactggtacattaaagccagcaattttcaaagatctcgattacgttgttaacgtctggagtaacggatgtttcgatttatgggaggaggtgaacggagttcatttctacacccttatggttatgagaaaagggctattgttgggggctgatttcgcgaagagaaacggtgactcaactagagcctcaacttactcttctactgcttccacaattgctaacaagatatcaagtttctgggttagctcaaacaactgggtgcaagtatcccaatctgtcacaggaggtgtaagtaaaaaggggttagacgttagcaccctgttagctgcgaatctaggatcagtcgatgatggatttttcactccaggttctgaaaagatattagctacagctgtggcagtcgaagattcctttgccagtctatacccaatcaacaaaaaccttccatcatacttggggaacgctattggaagataccctgaagatacatacaacggtaatggtaactcacaaggcaatccttggtttctggcggttaccggctacgcagagttgtactatagagcaattaaggaatggatttctaatggaggcgttacagtgtcctctatctcattgccatttttcaaaaagttcgatagctctgcaacatccggtaaaaagtacaccgtaggtacttctgacttcaacaatttagcacaaaacattgctcttgctgcagatcgtttcctatctactgtacaactccatgcaccaaacaatggttcattagcagaggaatttgatagaacaacaggtttttctaccggcgctagagatttaacatggtcccacgcctcattgataacagcatcctatgccaaagccggtgctccagctgcataattaattaaacaggccccttttcctttgtcgatatcatgtaattagttatgtcacgcttacattcacgccctcctcccacatccgctctaaccgaaaaggaaggagttagacaacctgaagtctaggtccctatttatttttttatagttatgttagtattaagaacgttatttatatttcaaatttttcttttttttctgtacaaacgcgtgtacgcatgtaacgggcagacggccggccataacttcgtataatgtatgctatacgaagttatccttacatcacacccaatcccccacaagtgatcccccacacaccatagcttcaaaatgtttctactccttttttactcttccagattttctcggactccgcgcatcgccgtaccacttcaaaacacccaagcacagcatactaaatttcccctctttcttcctctagggtggcgttaattacccgtactaaaggtttggaaaagaaaaaagagaccgcctcgtttctttttcttcgtcgaaaaaggcaataaaaatttttatcacgtttctttttcttgaaaaattttttttttgatttttttctctttcgatgacctcccattgatatttaagttaataaatggtcttcaatttctcaagtttcagtttcgtttttcttgttctattacaactttttttacttcttgctcattagaaagaaagcatagcaatctaatctaagttttaattacaaaatgccacaatcctgggaagaattggccgccgacaaacgtgcccgtttggctaaaaccattcctgacgaatggaaggttcaaactttgcctgccgaagattccgttattgatttcccaaagaagtccggtattttgtctgaggctgaattgaagattaccgaagcctctgctgctgatttggtctccaagttggccgctggtgagttgacttctgttgaagtcactttggctttttgtaagagagctgctattgctcaacaattaaccaactgtgctcacgaattcttcccagatgctgctttagctcaagctagagaattagatgaatactacgctaagcataagagaccagttggtccattacacggtttaccaatctctttaaaggaccaattgcgtgttaagggttacgaaacctccatgggttacatttcctggttaaacaaatacgatgaaggtgattccgtcttaaccaccatgttgagaaaagctggtgctgttttctacgttaagacctctgtcccacaaaccttgatggtctgtgaaaccgtcaacaacatcattggtagaactgtcaatccaagaaacaaaaattggtcctgtggtggttcttctggtggtgaaggtgctattgttggtattagaggtggtgttattggtgtcggtactgacattggtggttccattagagtcccagctgctttcaactttttatacggtttgagaccatctcacggtagattgccatatgctaaaatggctaactctatggaaggtcaagaaaccgttcactccgtcgttggtcctatcactcactccgtcgaagacttgagattgttcaccaaatctgtcttgggtcaagaaccttggaagtacgactctaaggtcatccccatgccatggagacaatctgaatctgacatcattgcctctaagattaagaatggtggtttgaacattggttattacaatttcgacggtaacgtcttgccacacccaccaattttacgtggtgtcgaaactaccgttgccgctttggc

SEQ ID NO: 19 - DNA, 5008 bp, synthetic construct
  misc_feature 1..5008: note = Mfa2-Rhizopus oryzae GA integration construct
  source 1..5008: mol_type = other DNA
ggccgcgaaggtgctattgttggtattagaggtggtgttattggtgtcggtactgacattggtggttccattagagtcccagctgctttcaactttttatacggtttgagaccatctcacggtagattgccatatgctaaaatggctaactctatggaaggtcaagaaaccgttcactccgtcgttggtcctatcactcactccgtcgaagacttgagattgttcaccaaatctgtcttgggtcaagaaccttggaagtacgactctaaggtcatcccaatgccatggagacaatctgaatctgacatcattgcctctaagattaagaatggtggtttgaacattggttattacaatttcgacggtaacgtcttgccacacccaccaattttacgtggtgtcgaaactaccgttgccgctttggccaaggctggtcacaccgttactccatggactccatacaagcatgatttcggtcatgacttgatttcccacatctatgctgctgatggttctgccgacgtcatgagagacatttctgcctctggtgagccagccatccctaacattaaggacttgttgaacccaaatattaaggctgttaacatgaacgaattgtgggacactcatttacaaaagtggaactatcaaatggaatacttggaaaagtggcgtgaagctgaagaaaaagctggtaaggaattggacgctattatcgctccaattactcctaccgccgctgtcagacacgatcaattcagatactacggttacgcctccgttattaacttattggatttcacctctgttgtcgtcccagtcactttcgctgataagaatattgataagaagaacgaatcttttaaagctgtttccgaattggatgctttggttcaagaagaatacgacccagaggcttatcacggtgctcctgttgctgttcaagttattggtagaagattgtccgaagagagaactttggctatcgccgaagaagtcggtaaattgttgggtaacgtcgtcactccataagcgaatttcttatgatttatgatttttattattaaataagttataaaaaaaataagtgtatacaaattttaaagtgactcttaggttttaaaacgaaaattcttattcttgagtaactctttcctgtaggtcaggttgctttctcaggtatagcatgaggtcgctcttattgaccacacctctaccggcatgccgagcaaatgcctgcaaatcgctccccatttcacccaattgtagatatgctaactccagcaatgagttgatgaatctcggtgtgtattttatgtcctcagaggacaacacataacttcgtataatgtatgctatacgaagttatctcgagggccagaaaaaggaagtgtttccctccttcttgaattgatgttaccctcataaagcacgtggcctcttatcgagaaagaaattaccgtcgctcgtgatttgtttgcaaaaagaacaaaactgaaaaaacccagacacgctcgacttcctgtcttcctgttgattgcagcttccaatttcgtcacacaacaaggtcctagcgacggctcacaggttttgtaacaagcaatcgaaggttctggaatggcgggaaagggtttagtaccacatgctatgatgcccactgtgatctccagagcaaagttcgttcgatcgtactgttactctctctctttcaaacagaattgtccgaatcgtgtgacaacaacagcctgttctcacacactcttttcttctaaccaagggggtggtttagtttagtagaacctcgtgaaacttacatttacatatatataaacttgcataaattggtcaatgcaagaaatacatatttggtcttttctaattcgtagtttttcaagttcttagatgctttctttttctcttttttacagatcatcaaggaagtaattatctactttttacaagtctagaatgaagtttatctccacgtttttaacctttatcctagcagctgtcagcgtcaccgccgcatcaattccgagttcagcatctgtacaacttgactcttacaattacgatggcagcactttctcagggaaaatttatgtgaaaaacatagcatatagtaagaaggttaccgtggtatatgcagacggttctgataattggaataataatggaaacactattgccgccagtttttccggcccaatttctggttccaattacgagtattggaccttttctgcatcagtaaaaggcatcaaggaattctatattaagtacgaagtttcaggtaagacatattacgataacaataactcagcaaattatcaagtctctacatctaagcccacaacaacaactgctgctaccaccactacaaccgctccttctaccagcaccactaccagaccaagctctagtgaaccggctacctttcctaccggaaacagtaccatctcaagctggatcaaaaagcaagaggacataagtcgttttgctatgttgaggaacattaatcctccaggatccgcgaccggtttcattgcagcatcactaagtactgccgggcctgattattattatgcttggactagagacgctgcattaacatcaaacgtgattgtttatgaatataatacgaccctttccggtaataaaacgatcttgaacgtattaaaagactatgtgacctttagtgtgaagacccaatctacatctacagtgtgtaattgtttgggagaacctaaattcaatccagacggttctgggtacactggtgcctggggtagacctcaaaacgacggtccagcagaaagagcaacaacctttgttctatttgctgactcttatttaacgcaaacaaaggacgcctcatatgttacagggaccctaaaaccagcaattttcaaagacttggattatgttgttaatgtttggagcaacggatgttttgacttgtgggaggaggttaacggtgtacacttttatacattgatggtgatgagaaaagggttgctattgggagcagatttcgctaaaagaaatggtgattctacaagagcgagcacatatagtagcaccgcttcaacaatcgccaataaaatctcatctttctgggtatctagcaacaactgggtacaagtttcccaaagtgttaccggcggtgtgtccaaaaagggtttagacgttagcacacttctagctgctaatttgggtagcgttgatgacgggttttttactccaggtagtgagaagatactggcaaccgcggtggcggttgaagacagctttgcttcattgtatcctataaataaaaatctgccctcttatctgggtaatgcaattggcagatacccagaagatacctacaatggtaatggtaattcccaggggaacccatggtttttggctgttacaggctacgcagaactttattaccgtgcaatcaaggaatggatttcaaatggcggcgtcactgtcagtagtataagtttgcccttttttaagaaatttgattcctcagcaacgtctggtaaaaaatacaccgtaggtactagtgatttcaataatttggcccaaaatattgcgcttgctgctgacaggtttcttagtaccgttcagttgcacgctccaaataatggctcattggctgaagaatttgatcgtacgacaggtttctccactggtgctagggatttgacttggagtcatgcctccttaatcacagcaagctatgctaaagctggtgcacctgctgcttagttaattaatttaccagcttactatccttcttgaaaatatgcactctatatcttttagttcttaattgcaacacatagatttgctgtataacgaattttatgctatttttttaatttggagttcggtgatgaaagtgtcacagcgaatttcctcacatgtagggaccgaattgtttacaagttctctgtaccaccatggagacatcaaagattgaaaatctatggaaagatatggacggtagcaacaagaatatagcacgagccgcggagttcatttcgttacttttgatatcgctcacaactattgcgaagcgcttcagtgaaaaaatcataaggaaaagttgtaaatattattggtagtattcgtttggtaaagtagagggggtaatttttcccctttattttgttcatacattcttaaattgctttgcctctccttttggaaagctatacttcggagcactgttgagcgaaggctcaggccggcagcacgcagcacgctgtatttacgtatttaattttatatatttgtgcatacactactagggaagacttgaaaaaaacctaggaaatgaaaaaacgacacaggaagtcccgtatttactattttttccttccttttgatggggcagggcggaaatagaggataggataagcctactgcttagctgtttccgtctctacttcggtagttgtctcaattgtcgtttcagtattacctttagagccgctagacgatggttgagctatttgttgagggaaaactaagttcatgtaacacacgcataacccgattaaactcatgaatagcttgattgcaggaggctggtccattggagatggtgccttattttccttataggcaacgatgatgtcttcgtcggtgttcaggtagtagtgtacactctgaatcagggagaaccaggcaatgaacttgttcctcaagaaaatagcggccataggcatggattggttaaccacaccagatatgcttggtgtggcagaatatagtccttttggtggcgcaattttcttgtacctgtggtagaaagggagcggttgaactgttagtatatattggcaatatcagcaaatttgaaagaaaattgtcggtgaaaaacatacgaaacacaaaggtcgggccttgcaacgttattcaaagtcattgtttagttgaggaggtagcagcggagtatatgtattccttttttttgcctatggatgttgtaccatgcccattctga

SEQ ID NO: 20 - DNA, 4884 bp, synthetic construct
  misc_feature 1..4884: note = Rhizopus microsporus GA integration construct
  source 1..4884: mol_type = other DNA
ctaaattcggccttgctcagagactcctggattttggctaacaacgcagtcccttcgatgcatatagctaggccacaaattatgccaataacggtccatgggttgatgttttcttgaattctttcgtttttcatgctatttgcgtcttcccaagtcccagcgttccagtattcatactgcgcgttagagtggtagccataagagccggcatattggtaattttcagtattaacgttagaacgtggtgaatacgatgtggtccagccttgcctcgttgtgtcatatacgatctttttctttgggtcacaaagaatatcatatgcttgagagatgactttaaatctatgtagtttttcgcttgatgttagcagcagcggtgatttactatcactgttggtaaccttttctgagctaaatatttgaatgttatcggaatggtcagggtggtacaattttacataacgatgatattttttttttaacgacttcttgtccagtttaggatttccagatccggcctttggaatgccaaaaatatcatagggagttggatctgccaactcaggccattgttcatcccttatcgtaagttttctattgccatttttatcgttcgctgtagcatacttagctataaaagtgatttgtgggggacacttttctacacatgataagtgccacttgaataaaaatgggtatacgaacttatggtgtagcataacaaatatattgcaagtagtgacctatggtgtgtagatatacgtacagttagttacgagcctaaagacacaacgtgtttgttaattatactgtcgctgtaatatcttctcttccattatcaccggtcattccttgcaggggcggtagtacccggagaccctgaacttttctttttttttttgcgaaattaaaaagttcattttcaattcgacaatgagatctacaagccattgttttatgttgatgagagccagcttaaagagttctcgagatctcccgagtttatcattatcaatactgccatttcaaagaatacgtaaataattaatagtagtgattttcctaactttatttagtcaaaaaattggccttttaattctgctgtaacccgtacatgcccaaaatagggggcgggttacacagaatatataacatcataggtgtctgggtgaacagtttattcctggcatccactaaatataatggagcccgctttttttaagctggcatccagaaaaaaaaagaatcccagcaccaaaatattgttttcttcaccaaccatcagttcataggtccattctcttagcgcaactacacagaacaggggcacaaacaggcaaaaaacgggcacaacctcaatggagtgatgcaacctgcttggagtaaatgatgacacaaggcaattgacctacgcatgtatctatctcattttcttacaccttctattaccttctgctctctctgatttggaaaaagctgaaaaaaaaggttgaaaccagttccctgaaattattcccctatttgactaataagtatataaagacggtaggtattgattgtaattctgtaaatctatttcttaaacttcttaaattctacttttatagttagtcttttttttagtttaaaacaccaagaacttagtttcgaataaacacacataaacaaacaaatctagaatgaaacttatgaatccatctatgaaggcatacgttttctttatcttaagctacttctctttactcgttagctcagctgcggtgccaacctctgccgccgtacaagttgagtcatacaattatgacggtaccactttttcaggtagaatattcgtcaaaaacattgcctactcaaaggtcgtaacagttatctactccgatggatcagataactggaacaataacaacaacaaagtttctgcagcttactcagaagcaatttctgggtctaactacgaatactggacattctccgcaaagttatccggaattaaacagttttatgtcaaatacgaagtttctggttcaacatattacgacaacaacggtaccaaaaactaccaagtccaagcaacctcagcgacatctacaacagctactgcaaccacaactacagctactggcacaacaactacttctacaggtccaactagtactgcatccgtatcattccctaccggtaactcaacaatttcttcctggataaaaaatcaagaggaaatcagccgttttgctatgttgagaaatatcaatccacctgggtctgccacagggttcatagccgcatctctgtccacagccggcccagattactattactcttggactagagattcagcactaacagctaatgtgatcgcttacgaatacaacacaacattcactggaaacaccacccttcttaagtacttgaaagattacgttacattttctgtcaaaagccaatctgtatctaccgtttgtaactgtctgggagaaccaaagttcaacgctgatggtagttcttttacaggtccatggggcagaccacaaaacgacggaccagcagagagagctgttacttttatgttgattgctgacagctacttgactcaaactaaggacgcatcctacgttaccggtacattaaagccagcaatcttcaaagatcttgattacgtagtttctgtttggtctaacggttgctacgatttatgggaagaggttaatggtgttcatttctatactctcatggtcatgagaaagggtttgatcttaggtgccgacttcgctgctagaaatggtgactctagtagagcttcaacctacaagcaaactgcatcaacaatggaatcaaagatcagttctttttggtcagattctaacaactacgtccaagtttctcaatcagttaccgccggagtgtcaaaaaagggactagatgttagtacactattggcggccaacattggtagtctgcctgatggctttttcactccaggctccgaaaagatattggctacagcagtggcgttagaaaatgcattcgcatccttgtacccaattaactctaacctaccttcttacttgggtaactcaattggaagatatcctgaggatacatacaacggtaatggcaactctcaggggaatccatggttccttgccgtcaacgcatacgcagaactttactacagagctattaaggaatggattagtaatggcaaggtgacagtatccaatatctcactacctttcttcaaaaagtttgattcttccgccacttctggaaagacatacactgctggtacatcagatttcaataacttggctcagaacattgctttaggcgccgatagattcctgtctactgttaagttccacgcatacactaacgggagtctatcagaagagtacgatagatctaccggtatgagtactggggctcgtgatttaacatggtcccatgcttcattgatcacagtggcgtacgcaaaggccggtagtcctgcagcttagttaattaaacaggccccttttcctttgtcgatatcatgtaattagttatgtcacgcttacattcacgccctcctcccacatccgctctaaccgaaaaggaaggagttagacaacctgaagtctaggtccctatttatttttttatagttatgttagtattaagaacgttatttatatttcaaatttttcttttttttctgtacaaacgcgtgtacgcatgtaacgggcagacggccggccataacttcgtataatgtatgctatacgaagttatggcaacggttcatcatctcatggatctgcacatgaacaaacaccagagtcaaacgacgttgaaattgaggctactgcgccaattgatgacaatacagacgatgataacaaaccgaagttatctgatgtagaaaaggattagagatgctaagagatagtgatgatatttcataaataatgtaattctatatatgttaattaccttttttgcgaggcatatttatggtgaaggataagttttgaccatcaaagaaggttaatgtggctgtggtttcagggtccataaagcttttcaattcatcttttttttttttgttcttttttttgattccggtttctttgaaatttttttgattcggtaatctccgagcagaaggaagaacgaaggaaggagcacagacttagattggtatatatacgcatatgtggtgttgaagaaacatgaaattgcccagtattcttaacccaactgcacagaacaaaaacctgcaggaaacgaagataaatcatgtcgaaagctacatataaggaacgtgctgctactcatcctagtcctgttgctgccaagctatttaatatcatgcacgaaaagcaaacaaacttgtgtgcttcattggatgttcgtaccaccaaggaattactggagttagttgaagcattaggtcccaaaatttgtttactaaaaacacatgtggatatcttgactgatttttccatggagggcacagttaagccgctaaaggcattatccgccaagtacaattttttactcttcgaagacagaaaatttgctgacattggtaatacagtcaaattgcagtactctgcgggtgtatacagaatagcagaatgggcagacattacgaatgcacacggtgtggtgggcccaggtattgttagcggtttgaagcaggcggcggaagaagtaacaaaggaacctagaggccttttgatgttagcagaattgtcatgcaagggctccctagctactggagaatatactaagggtactgttgacattgcgaagagcgacaaagattttgttatcggctttattgctcaaagagacatgggtggaagagatgaaggttacgattggttgattatgacacgc

SEQ ID NO: 21 - DNA, 1790 bp, synthetic construct
  misc_feature 1..1790: note = Integration construct
  source 1..1790: mol_type = other DNA
ggaagagctcctactgcgccaattgatgacaatacagacgatgataacaaaccgaagttatctgatgtagaaaaggattagagatgctaagagatagtgatgatatttcataaataatgtaattctatatatgttaattaccttttttgcgaggcatatttatggtgaaggataagttttgaccatcaaagaaggttaatgtggctgtggtttcagggtccataaagcttttcaattcatctttttttttttgttcttttttttgattccggtttctttgaaatttttttgattcggtaatctccgagcagaaggaagaacgaaggaaggagcacagacttagattggtatatatacgcatatgtggtgttgaagaaacatgaaattgcccagtattcttaacccaactgcacagaacaaaaacctgcaggaaacgaagataaatcatgtcgaaagctacatataaggaacgtgctgctactcatcctagtcctgttgctgccaagctatttaatatcatgcacgaaaagcaaacaaacttgtgtgcttcattggatgttcgtaccaccaaggaattactggagttagttgaagcattaggtcccaaaatttgtttactaaaaacacatgtggatatcttgactgatttttccatggagggcacagttaagccgctaaaggcattatccgccaagtacaattttttactcttcgaagacagaaaatttgctgacattggtaatacagtcaaattgcagtactctgcgggtgtatacagaatagcagaatgggcagacattacgaatgcgcacggtgtggtgggcccaggtattgttagcggtttgaagcaggcggcggaagaagtaacaaaggaacctagaggccttttgatgttagcagaattgtcatgcaagggctccctagctactggagaatatactaagggtactgttgacattgcgaagagcgacaaagattttgttatcggctttattgctcaaagagacatgggtggaagagatgaaggttacgattggttgattatgacacccggtgtgggtttagatgacaagggagacgcattgggtcaacagtatagagccgtggatgatgtggtctctacaggatctgacattattattgttggaagaggactatttgcaaagggaagggatgctaaggtagagggtgaacgttacagaaaagcaggctgggaagcatatttgagaagatgcggccagcaaaactaaaaaactgtattataagtaaatgcatgtatactaaactcacaaattagagcttcaatttaattatatcagttattacccgggaatctcggtcgtaatgatttttataatgacgaaaaaaaaaaattggaaagaaaaagcttcatggcctttataaaaaggaaccatccaatacctcgccagaaccaagtaacagtattttacggggcacaaatcaagaacaataagacaggactgtaaagatggacgcattgaactccaaagaacaacaagagttccaaaaagtagtggaacaaaagcaaatgaaggatttcatgcgtttgataacttcgtataatgtatgctatacgaagttatgcggccgccagcacgcagcacgctgtatttacgtatttaattttatatatttgtgcatacactactagggaagacttgaaaaaaacctaggaaatgaaaaaacgacacaggaagtcccgtatttactattttttccttccttttgatggggcagggcggaaatagaggataggataagcctactgc

SEQ ID NO: 22 - DNA, 4474 bp, synthetic construct
  misc_feature 1..4474: note = Rhizopus microsporus GA integration construct
  source 1..4474: mol_type = other DNA
gtgtttgttaattatactgtcgctgtaatatcttctcttccattatcaccggtcattccttgcaggggcggtagtacccggagaccctgaacttttctttttttttttgcgaaattaaaaagttcattttcaattcgacaatgagatctacaagccattgttttatgttgatgagagccagcttaaagagttctcgagatctcccgagtttatcattatcaatactgccatttcaaagaatacgtaaataattaatagtagtgattttcctaactttatttagtcaaaaaattggccttttaattctgctgtaacccgtacatgcccaaaatagggggcgggttacacagaatatataacatcataggtgtctgggtgaacagtttattcctggcatccactaaatataatggagcccgctttttttaagctggcatccagaaaaaaaaagaatcccagcaccaaaatattgttttcttcaccaaccatcagttcataggtccattctcttagcgcaactacacagaacaggggcacaaacaggcaaaaaacgggcacaacctcaatggagtgatgcaacctgcttggagtaaatgatgacacaaggcaattgacctacgcatgtatctatctcattttcttacaccttctattaccttctgctctctctgatttggaaaaagctgaaaaaaaaggttgaaaccagttccctgaaattattcccctatttgactaataagtatataaagacggtaggtattgattgtaattctgtaaatctatttcttaaacttcttaaattctacttttatagttagtcttttttttagtttaaaacaccaagaacttagtttcgaataaacacacataaacaaacaaatctagaatgaaacttatgaatccatctatgaaggcatacgttttctttatcttaagctacttctctttactcgttagctcagctgcggtgccaacctctgccgccgtacaagttgagtcatacaattatgacggtaccactttttcaggtagaatattcgtcaaaaacattgcctactcaaaggtcgtaacagttatctactccgatggatcagataactggaacaataacaacaacaaagtttctgcagcttactcagaagcaatttctgggtctaactacgaatactggacattctccgcaaagttatccggaattaaacagttttatgtcaaatacgaagtttctggttcaacatattacgacaacaacggtaccaaaaactaccaagtccaagcaacctcagcgacatctacaacagctactgcaaccacaactacagctactggcacaacaactacttctacaggtccaactagtactgcatccgtatcattccctaccggtaactcaacaatttcttcctggataaaaaatcaagaggaaatcagccgttttgctatgttgagaaatatcaatccacctgggtctgccacagggttcatagccgcatctctgtccacagccggcccagattactattactcttggactagagattcagcactaacagctaatgtgatcgcttacgaatacaacacaacattcactggaaacaccacccttcttaagtacttgaaagattacgttacattttctgtcaaaagccaatctgtatctaccgtttgtaactgtctgggagaaccaaagttcaacgctgatggtagttcttttacaggtccatggggcagaccacaaaacgacggaccagcagagagagctgttacttttatgttgattgctgacagctacttgactcaaactaaggacgcatcctacgttaccggtacattaaagccagcaatcttcaaagatcttgattacgtagtttctgtttggtctaacggttgctacgatttatgggaagaggttaatggtgttcatttctatactctcatggtcatgagaaagggtttgatcttaggtgccgacttcgctgctagaaatggtgactctagtagagcttcaacctacaagcaaactgcatcaacaatggaatcaaagatcagttctttttggtcagattctaacaactacgtccaagtttctcaatcagttaccgccggagtgtcaaaaaagggactagatgttagtacactattggcggccaacattggtagtctgcctgatggctttttcactccaggctccgaaaagatattggctacagcagtggcgttagaaaatgcattcgcatccttgtacccaattaactctaacctaccttcttacttgggtaactcaattggaagatatcctgaggatacatacaacggtaatggcaactctcaggggaatccatggttccttgccgtcaacgcatacgcagaactttactacagagctattaaggaatggattagtaatggcaaggtgacagtatccaatatctcactacctttcttcaaaaagtttgattcttccgccacttctggaaagacatacactgctggtacatcagatttcaataacttggctcagaacattgctttaggcgccgatagattcctgtctactgttaagttccacgcatacactaacgggagtctatcagaagagtacgatagatctaccggtatgagtactggggctcgtgatttaacatggtcccatgcttcattgatcacagtggcgtacgcaaaggccggtagtcctgcagcttagttaattaaacaggccccttttcctttgtcgatatcatgtaattagttatgtcacgcttacattcacgccctcctcccacatccgctctaaccgaaaaggaaggagttagacaacctgaagtctaggtccctatttatttttttatagttatgttagtattaagaacgttatttatatttcaaatttttcttttttttctgtacaaacgcgtgtacgcatgtaacgggcagacggccggccataacttcgtataatgtatgctatacgaagttatccttacatcacacccaatcccccacaagtgatcccccacacaccatagcttcaaaatgtttctactccttttttactcttccagattttctcggactccgcgcatcgccgtaccacttcaaaacacccaagcacagcatactaaatttcccctctttcttcctctagggtggcgttaattacccgtactaaaggtttggaaaagaaaaaagagaccgcctcgtttctttttcttcgtcgaaaaaggcaataaaaatttttatcacgtttctttttcttgaaaaattttttttttgatttttttctctttcgatgacctcccattgatatttaagttaataaatggtcttcaatttctcaagtttcagtttcgtttttcttgttctattacaactttttttacttcttgctcattagaaagaaagcatagcaatctaatctaagttttaattacaaaatgccacaatcctgggaagaattggccgccgacaaacgtgcccgtttggctaaaaccattcctgacgaatggaaggttcaaactttgcctgccgaagattccgttattgatttcccaaagaagtccggtattttgtctgaggctgaattgaagattaccgaagcctctgctgctgatttggtctccaagttggccgctggtgagttgacttctgttgaagtcactttggctttttgtaagagagctgctattgctcaacaattaaccaactgtgctcacgaattcttcccagatgctgctttagctcaagctagagaattagatgaatactacgctaagcataagagaccagttggtccattacacggtttaccaatctctttaaaggaccaattgcgtgttaagggttacgaaacctccatgggttacatttcctggttaaacaaatacgatgaaggtgattccgtcttaaccaccatgttgagaaaagctggtgctgttttctacgttaagacctctgtcccacaaaccttgatggtctgtgaaaccgtcaacaacatcattggtagaactgtcaatccaagaaacaaaaattggtcctgtggtggttcttctggtggtgaaggtgctattgttggtattagaggtggtgttattggtgtcggtactgacattggtggttccattagagtcccagctgctttcaactttttatacggtttgagaccatctcacggtagattgccatatgctaaaatggctaactctatggaaggtcaagaaaccgttcactccgtcgttggtcctatcactcactccgtcgaagacttgagattgttcaccaaatctgtcttgggtcaagaaccttggaagtacgactctaaggtcatccccatgccatggagacaatctgaatctgacatcattgcctctaagattaagaatggtggtttgaacattggttattacaatttcgacggtaacgtcttgccacacccaccaattttacgtggtgtcgaaactaccgttgccgctttggc

SEQ ID NO: 23 - DNA, 1878 bp, synthetic construct
  misc_feature 1..1878: note = Integration construct
  source 1..1878: mol_type = other DNA
gaagattaccgaagcctctgctgctgatttggtctccaagttggccgctggtgagttgacttctgttgaagtcactttggctttttgtaagagagctgctattgctcaacaattaaccaactgtgctcacgaattcttcccagatgctgctttagctcaagctagagaattagatgaatactacgctaagcataagagaccagttggtccattacacggtttaccaatctctttaaaggaccaattgcgtgttaagggttacgaaacctccatgggttacatttcctggttaaacaaatacgatgaaggtgattccgtcttaaccaccatgttgagaaaagctggtgctgttttctacgttaagacctctgtcccacaaaccttgatggtctgtgaaaccgtcaacaacatcattggtagaactgtcaatccaagaaacaaaaattggtcctgtggtggttcttctggtggtgaaggtgctattgttggtattagaggtggtgttattggtgtcggtactgacattggtggttccattagagtcccagctgctttcaactttttatacggtttgagaccatctcacggtagattgccatatgctaaaatggctaactctatggaaggtcaagaaaccgttcactccgtcgttggtcctatcactcactccgtcgaagacttgagattgttcaccaaatctgtcttgggtcaagaaccttggaagtacgactctaaggtcatcccaatgccatggagacaatctgaatctgacatcattgcctctaagattaagaatggtggtttgaacattggttattacaatttcgacggtaacgtcttgccacacccaccaattttacgtggtgtcgaaactaccgttgccgctttggccaaggctggtcacaccgttactccatggactccatacaagcatgatttcggtcatgacttgatttcccacatctatgctgctgatggttctgccgacgtcatgagagacatttctgcctctggtgagccagccatccctaacattaaggacttgttgaacccaaatattaaggctgttaacatgaacgaattgtgggacactcatttacaaaagtggaactatcaaatggaatacttggaaaagtggcgtgaagctgaagaaaaagctggtaaggaattggacgctattatcgctccaattactcctaccgccgctgtcagacacgatcaattcagatactacggttacgcctccgttattaacttattggatttcacctctgttgtcgtcccagtcactttcgctgataagaatattgataagaagaacgaatcttttaaagctgtttccgaattggatgctttggttcaagaagaatacgacccagaggcttatcacggtgctcctgttgctgttcaagttattggtagaagattgtccgaagagagaactttggctatcgccgaagaagtcggtaaattgttgggtaacgtcgtcactccataaggagattgataagacttttctagttgcatatcttttatatttaaatcttatctattagttaattttttgtaatttatccttatatatagtctggttattctaaaatatcatttcagtatctaaaaattcccctcttttttcagttatatcttaacaggcgataacttcgtataatgtatgctatacgaagttatgcggccgccagcacgcagcacgctgtatttacgtatttaattttatatatttgtgcatacactactagggaagacttgaaaaaaacctaggaaatgaaaaaacgacacaggaagtcccgtatttactattttttccttccttttgatggggcagggcggaaatagaggataggataagcctactgc

SEQ ID NO: 24 - DNA, 4827 bp, synthetic construct
  misc_feature 1..4827: note = Rhizopus microsporus GA integration construct
  source 1..4827: mol_type = other DNA
ggccgctccatggagggcacagttaagccgctaaaggcattatccgccaagtacaattttttactcttcgaagacagaaaatttgctgacattggtaatacagtcaaattgcagtactctgcgggtgtatacagaatagcagaatgggcagacattacgaatgcacacggtgtggtgggcccaggtattgttagcggtttgaagcaggcggcggaagaagtaacaaaggaacctagaggccttttgatgttagcagaattgtcatgcaagggctccctagctactggagaatatactaagggtactgttgacattgcgaagagcgacaaagattttgttatcggctttattgctcaaagagacatgggtggaagagatgaaggttacgattggttgattatgacacccggtgtgggtttagatgacaagggagacgcattgggtcaacagtatagaaccgtggatgatgtggtctctacaggatctgacattattattgttggaagaggactatttgcaaagggaagggatgctaaggtagagggtgaacgttacagaaaagcaggctgggaagcatatttgagaagatgcggccagcaaaactaaaaaactgtattataagtaaatgcatgtatactaaactcacaaattagagcttcaatttaattatatcagttattacccgggaatctcggtcgtaatgatttttataatgacgaaaaaaaaaaaattggaaagaaaaagcttcatggcctttataaaaaggaaccatccaatacctcgccagaaccaagtaacagtattttacggggcacaaatcaagaacaataagacaggactgtaaagatggacgcattgaactccaaagaacaacaagagttccaaaaagtagtggaacaaaagcaaatgaaggatttcatgcgtttgataacttcgtataatgtatgctatacgaagttatctcgagggccagaaaaaggaagtgtttccctccttcttgaattgatgttaccctcataaagcacgtggcctcttatcgagaaagaaattaccgtcgctcgtgatttgtttgcaaaaagaacaaaactgaaaaaacccagacacgctcgacttcctgtcttcctgttgattgcagcttccaatttcgtcacacaacaaggtcctagcgacggctcacaggttttgtaacaagcaatcgaaggttctggaatggcgggaaagggtttagtaccacatgctatgatgcccactgtgatctccagagcaaagttcgttcgatcgtactgttactctctctctttcaaacagaattgtccgaatcgtgtgacaacaacagcctgttctcacacactcttttcttctaaccaagggggtggtttagtttagtagaacctcgtgaaacttacatttacatatatataaacttgcataaattggtcaatgcaagaaatacatatttggtcttttctaattcgtagtttttcaagttcttagatgctttctttttctcttttttacagatcatcaaggaagtaattatctactttttacaagtctagaatgaagctaatgaacccatctatgaaagcttatgtctttttcatcttatcatacttctctctcctagtttcatctgccgcagtgcctacatctgctgccgtccaagtggaaagttacaattacgatggcactaccttctccggccgtatcttcgtgaaaaacattgcttactcaaaagttgttacagtgatttactccgatggttctgataattggaacaacaataacaacaaagtttcagcagcgtactccgaagccattagtggatctaactacgaatactggactttctccgcaaagttgtctggtattaagcaattctacgtaaagtacgaagtttcaggttcaacatactacgataacaatggtactaaaaactaccaggtacaagccacaagcgctacaagtacaactgccacagctacaactacaactgctacagggacaacaactacatcaaccggtccaacatcaaccgcatctgtctcctttccaaccggtaacagtacaatatcatcatggatcaaaaaccaagaggaaatctcaagatttgcaatgttgagaaacatcaatccaccagggtcagcgactggtttcatcgccgcttcattgtccaccgctgggccagactactattactcttggactagagactctgcattgacagcaaacgttatagcttacgaatacaacacaaccttcactggtaacactaccttgttgaagtatcttaaagactacgtcacttttagtgttaagtctcaatctgtttctaccgtctgtaactgtttaggtgaaccaaagtttaatgcagatggctcatcatttactggtccatggggcagacctcaaaacgatggaccagcagaaagagcagtcacattcatgttgatcgctgactcatacttgacacaaactaaggatgcttcatacgtgactggaacactcaagccagccatattcaaagacctggattatgttgtttctgtgtggtctaatggttgctacgatttgtgggaggaagttaatggcgtacatttctacacactaatggttatgagaaagggactaattcttggggcagatttcgcagctagaaatggtgattcctcaagagcatctacctacaagcaaacagcatctacaatggaatcaaagatcagctctttctggtctgactctaacaactacgttcaagtttcacaatctgtgactgctggtgtaagtaaaaagggtttagatgtttctactctgttagctgcaaacattggttctttaccagatggcttctttacaccaggatcagaaaagattttggcaactgccgttgccttagagaatgcattcgcttccctttaccctattaactctaacttaccttcatatttgggtaattcaattggtagatatccagaggacacatacaacggaaacgggaattcacagggcaacccttggttcttagccgtaaacgcgtacgccgagttatactacagagccattaaggaatggatctcaaatggtaaggtaacagtctctaatatctctcttcctttctttaaaaagttcgattctagcgccactagcggcaagacctatacagccggaacaagtgatttcaataacctcgctcagaacatagctcttggagcagacagatttctgtcaactgttaaatttcacgcgtacacaaatggcagcttgtctgaagagtacgatcgttccaccgggatgagtactggtgctagagatctaacctggtcccatgcatctcttatcacagttgcatacgcaaaagctggatctcctgctgcgtaattaattaatttaccagcttactatccttcttgaaaatatgcactctatatcttttagttcttaattgcaacacatagatttgctgtataacgaattttatgctatttttttaatttggagttcggtgatgaaagtgtcacagcgaatttcctcacatgtagggaccgaattgtttacaagttctctgtaccaccatggagacatcaaagattgaaaatctatggaaagatatggacggtagcaacaagaatatagcacgagccgcggagttcatttcgttacttttgatatcgctcacaactattgcgaagcgcttcagtgaaaaaatcataaggaaaagttgtaaatattattggtagtattcgtttggtaaagtagagggggtaatttttcccctttattttgttcatacattcttaaattgctttgcctctccttttggaaagctatacttcggagcactgttgagcgaaggctcaggccggcagcacgcagcacgctgtatttacgtatttaattttatatatttgtgcatacactactagggaagacttgaaaaaaacctaggaaatgaaaaaacgacacaggaagtcccgtatttactattttttccttccttttgatggggcagggcggaaatagaggataggataagcctactgcttagctgtttccgtctctacttcggtagttgtctcaattgtcgtttcagtattacctttagagccgctagacgatggttgagctatttgttgagggaaaactaagttcatgtaacacacgcataacccgattaaactcatgaatagcttgattgcaggaggctggtccattggagatggtgccttattttccttataggcaacgatgatgtcttcgtcggtgttcaggtagtagtgtacactctgaatcagggagaaccaggcaatgaacttgttcctcaagaaaatagcggccataggcatggattggttaaccacaccagatatgcttggtgtggcagaatatagtccttttggtggcgcaattttcttgtacctgtggtagaaagggagcggttgaactgttagtatatattggcaatatcagcaaatttgaaagaaaattgtcggtgaaaaacatacgaaacacaaaggtcgggccttgcaacgttattcaaagtcattgtttagttgaggaggtagcagcggagtatatgtattccttttttttgcctatggatgttgtaccatgcccattctgctcaagcttttgttaaaattatttttcagtattttttcttccatgttgcgcgttacgagaacagaagcgacagataaccgcaatcatacaactagcgctactgcggggtgtaaaaagcacaagaactaagccaagatcacaacagttatcgataaaatagcagtgtttgcatggccattgagaaggacaacattggcgtgcggcatg

SEQ ID NO: 25 - DNA, 4684 bp, synthetic construct
  misc_feature 1..4684: note = Rhizopus microsporus GA integration construct
  source 1..4684: mol_type = other DNA
ggccgcgaaggtgctattgttggtattagaggtggtgttattggtgtcggtactgacattggtggttccattagagtcccagctgctttcaactttttatacggtttgagaccatctcacggtagattgccatatgctaaaatggctaactctatggaaggtcaagaaaccgttcactccgtcgttggtcctatcactcactccgtcgaagacttgagattgttcaccaaatctgtcttgggtcaagaaccttggaagtacgactctaaggtcatcccaatgccatggagacaatctgaatctgacatcattgcctctaagattaagaatggtggtttgaacattggttattacaatttcgacggtaacgtcttgccacacccaccaattttacgtggtgtcgaaactaccgttgccgctttggccaaggctggtcacaccgttactccatggactccatacaagcatgatttcggtcatgacttgatttcccacatctatgctgctgatggttctgccgacgtcatgagagacatttctgcctctggtgagccagccatccctaacattaaggacttgttgaacccaaatattaaggctgttaacatgaacgaattgtgggacactcatttacaaaagtggaactatcaaatggaatacttggaaaagtggcgtgaagctgaagaaaaagctggtaaggaattggacgctattatcgctccaattactcctaccgccgctgtcagacacgatcaattcagatactacggttacgcctccgttattaacttattggatttcacctctgttgtcgtcccagtcactttcgctgataagaatattgataagaagaacgaatcttttaaagctgtttccgaattggatgctttggttcaagaagaatacgacccagaggcttatcacggtgctcctgttgctgttcaagttattggtagaagattgtccgaagagagaactttggctatcgccgaagaagtcggtaaattgttgggtaacgtcgtcactccataagcgaatttcttatgatttatgatttttattattaaataagttataaaaaaaataagtgtatacaaattttaaagtgactcttaggttttaaaacgaaaattcttattcttgagtaactctttcctgtaggtcaggttgctttctcaggtatagcatgaggtcgctcttattgaccacacctctaccggcatgccgagcaaatgcctgcaaatcgctccccatttcacccaattgtagatatgctaactccagcaatgagttgatgaatctcggtgtgtattttatgtcctcagaggacaacacataacttcgtataatgtatgctatacgaagttatctcgagggccagaaaaaggaagtgtttccctccttcttgaattgatgttaccctcataaagcacgtggcctcttatcgagaaagaaattaccgtcgctcgtgatttgtttgcaaaaagaacaaaactgaaaaaacccagacacgctcgacttcctgtcttcctgttgattgcagcttccaatttcgtcacacaacaaggtcctagcgacggctcacaggttttgtaacaagcaatcgaaggttctggaatggcgggaaagggtttagtaccacatgctatgatgcccactgtgatctccagagcaaagttcgttcgatcgtactgttactctctctctttcaaacagaattgtccgaatcgtgtgacaacaacagcctgttctcacacactcttttcttctaaccaagggggtggtttagtttagtagaacctcgtgaaacttacatttacatatatataaacttgcataaattggtcaatgcaagaaatacatatttggtcttttctaattcgtagtttttcaagttcttagatgctttctttttctcttttttacagatcatcaaggaagtaattatctactttttacaagtctagaatgaagctaatgaacccatctatgaaagcttatgtctttttcatcttatcatacttctctctcctagtttcatctgccgcagtgcctacatctgctgccgtccaagtggaaagttacaattacgatggcactaccttctccggccgtatcttcgtgaaaaacattgcttactcaaaagttgttacagtgatttactccgatggttctgataattggaacaacaataacaacaaagtttcagcagcgtactccgaagccattagtggatctaactacgaatactggactttctccgcaaagttgtctggtattaagcaattctacgtaaagtacgaagtttcaggttcaacatactacgataacaatggtactaaaaactaccaggtacaagccacaagcgctacaagtacaactgccacagctacaactacaactgctacagggacaacaactacatcaaccggtccaacatcaaccgcatctgtctcctttccaaccggtaacagtacaatatcatcatggatcaaaaaccaagaggaaatctcaagatttgcaatgttgagaaacatcaatccaccagggtcagcgactggtttcatcgccgcttcattgtccaccgctgggccagactactattactcttggactagagactctgcattgacagcaaacgttatagcttacgaatacaacacaaccttcactggtaacactaccttgttgaagtatcttaaagactacgtcacttttagtgttaagtctcaatctgtttctaccgtctgtaactgtttaggtgaaccaaagtttaatgcagatggctcatcatttactggtccatggggcagacctcaaaacgatggaccagcagaaagagcagtcacattcatgttgatcgctgactcatacttgacacaaactaaggatgcttcatacgtgactggaacactcaagccagccatattcaaagacctggattatgttgtttctgtgtggtctaatggttgctacgatttgtgggaggaagttaatggcgtacatttctacacactaatggttatgagaaagggactaattcttggggcagatttcgcagctagaaatggtgattcctcaagagcatctacctacaagcaaacagcatctacaatggaatcaaagatcagctctttctggtctgactctaacaactacgttcaagtttcacaatctgtgactgctggtgtaagtaaaaagggtttagatgtttctactctgttagctgcaaacattggttctttaccagatggcttctttacaccaggatcagaaaagattttggcaactgccgttgccttagagaatgcattcgcttccctttaccctattaactctaacttaccttcatatttgggtaattcaattggtagatatccagaggacacatacaacggaaacgggaattcacagggcaacccttggttcttagccgtaaacgcgtacgccgagttatactacagagccattaaggaatggatctcaaatggtaaggtaacagtctctaatatctctcttcctttctttaaaaagttcgattctagcgccactagcggcaagacctatacagccggaacaagtgatttcaataacctcgctcagaacatagctcttggagcagacagatttctgtcaactgttaaatttcacgcgtacacaaatggcagcttgtctgaagagtacgatcgttccaccgggatgagtactggtgctagagatctaacctggtcccatgcatctcttatcacagttgcatacgcaaaagctggatctcctgctgcgtaattaattaatttaccagcttactatccttcttgaaaatatgcactctatatcttttagttcttaattgcaacacatagatttgctgtataacgaattttatgctatttttttaatttggagttcggtgatgaaagtgtcacagcgaatttcctcacatgtagggaccgaattgtttacaagttctctgtaccaccatggagacatcaaagattgaaaatctatggaaagatatggacggtagcaacaagaatatagcacgagccgcggagttcatttcgttacttttgatatcgctcacaactattgcgaagcgcttcagtgaaaaaatcataaggaaaagttgtaaatattattggtagtattcgtttggtaaagtagagggggtaatttttcccctttattttgttcatacattcttaaattgctttgcctctccttttggaaagctatacttcggagcactgttgagcgaaggctcaggccggcagcacgcagcacgctgtatttacgtatttaattttatatatttgtgcatacactactagggaagacttgaaaaaaacctaggaaatgaaaaaacgacacaggaagtcccgtatttactattttttccttccttttgatggggcagggcggaaatagaggataggataagcctactgcttagctgtttccgtctctacttcggtagttgtctcaattgtcgtttcagtattacctttagagccgctagacgatggttgagctatttgttgagggaaaactaagttcatgtaacacacgcataacccgattaaactcatgaatagcttgattgcaggaggctggtccattggagatggtgccttattttccttataggcaacgatgatgtcttcgtcggtgttcaggtagtagt

SEQ ID NO: 26 - DNA, 4909 bp, synthetic construct
  misc_feature 1..4909: note = Rhizopus delemar GA integration construct
  source 1..4909: mol_type = other DNA
ctaaattcggccttgctcagagactcctggattttggctaacaacgcagtcccttcgatgcatatagctaggccacaaattatgccaataacggtccatgggttgatgttttcttgaattctttcgtttttcatgctatttgcgtcttcccaagtcccagcgttccagtattcatactgcgcgttagagtggtagccataagagccggcatattggtaattttcagtattaacgttagaacgtggtgaatacgatgtggtccagccttgcctcgttgtgtcatatacgatctttttctttgggtcacaaagaatatcatatgcttgagagatgactttaaatctatgtagtttttcgcttgatgttagcagcagcggtgatttactatcactgttggtaaccttttctgagctaaatatttgaatgttatcggaatggtcagggtggtacaattttacataacgatgatattttttttttaacgacttcttgtccagtttaggatttccagatccggcctttggaatgccaaaaatatcatagggagttggatctgccaactcaggccattgttcatcccttatcgtaagttttctattgccatttttatcgttcgctgtagcatacttagctataaaagtgatttgtgggggacacttttctacacatgataagtgccacttgaataaaaatgggtatacgaacttatggtgtagcataacaaatatattgcaagtagtgacctatggtgtgtagatatacgtacagttagttacgagcctaaagacacaacgtgtttgttaattatactgtcgctgtaatatcttctcttccattatcaccggtcattccttgcaggggcggtagtacccggagaccctgaacttttctttttttttttgcgaaattaaaaagttcattttcaattcgacaatgagatctacaagccattgttttatgttgatgagagccagcttaaagagttctcgagatctcccgagtttatcattatcaatactgccatttcaaagaatacgtaaataattaatagtagtgattttcctaactttatttagtcaaaaaattggccttttaattctgctgtaacccgtacatgcccaaaatagggggcgggttacacagaatatataacatcataggtgtctgggtgaacagtttattcctggcatccactaaatataatggagcccgctttttttaagctggcatccagaaaaaaaaagaatcccagcaccaaaatattgttttcttcaccaaccatcagttcataggtccattctcttagcgcaactacacagaacaggggcacaaacaggcaaaaaacgggcacaacctcaatggagtgatgcaacctgcttggagtaaatgatgacacaaggcaattgacctacgcatgtatctatctcattttcttacaccttctattaccttctgctctctctgatttggaaaaagctgaaaaaaaaggttgaaaccagttccctgaaattattcccctatttgactaataagtatataaagacggtaggtattgattgtaattctgtaaatctatttcttaaacttcttaaattctacttttatagttagtcttttttttagtttaaaacaccaagaacttagtttcgaataaacacacataaacaaacaaatctagaatgcagttattcaacttaccacttaaggtatctttctttctagtcttatcttacttttcattgttagtatcagctgcctctataccaagttcagcatccgtacaactagattcatacaattacgacggttcaacattctcaggaaagatatacgtgaaaaatattgcttacagcaaaaaggttactgtgatttacgcagatgggtcagacaactggaataacaatggaaacacaattgctgcttcctattctgcccctatttctggatctaactacgaatactggactttttcagcgagtataaacggaattaaggaattctatatcaaatatgaagtctctggtaagacctactacgataacaacaactccgcaaactaccaagttagcacatcaaagccaaccacaacaactgctactgcgacaactacaaccgcaccaagcacttctactacaacacctcctagttcatctgagccagcaactttcccaactggtaattccactatttcttcttggatcaaaaaacaagagggtatctcaagattcgccatgcttagaaatatcaatcctccaggctctgcaacaggattcattgcagcatctttatcaactgcggggccagactactactacgcctggactagagatgcagctttgacatcaaatgtgattgtttatgaatacaacacaactttgtccggtaacaagacaatcttgaacgtcttgaaggattatgtgacattctctgtcaagactcaatctacatcaacagtttgtaactgtctcggcgaaccaaagttcaaccctgatggtagtggttacactggtgcttggggtagaccacaaaacgatggtccagcagagagagctacaactttcatcttgtttgctgactcttacctaacacaaaccaaggatgcaagctacgttactggaacactaaagcctgcaatctttaaagacctggactatgttgtaaacgtttggtcaaatggctgcttcgatctatgggaggaagtgaacggtgttcacttctacacattaatggtcatgagaaagggactcttgcttggtgcagactttgctaagagaaacggtgattctacacgtgcctccacttactcctccacagcttcaaccattgccaacaaaatctcttctttctgggtcagctcaaataactggattcaagtttctcaatcagttactggtggtgtttctaaaaagggcctggatgtgtcaaccttgcttgctgccaatttgggcagtgttgatgacgggttcttcaccccaggttctgaaaagatcctcgccaccgcagttgccgttgaagattcatttgctagtttatacccaatcaacaaaaatctaccatcataccttggaaattcaatcggtagatatccagaggatacatacaacggtaatggaaactctcagggtaacccttggtttcttgcagttacagggtacgctgaactgtactacagagcgattaaggaatggattggtaatggcggcgtaactgttagttctatttctctacctttcttcaaaaagttcgatagttctgcaacatctggtaaaaagtacacagtcggcacttccgattttaacaatttagctcagaacatagcactggcagctgatcgtttcttgagtacagtccaattgcatgcccataacaacggtagtttggctgaagagtttgatagaaccaccggtttatcaaccggcgccagagatttaacatggtcccatgcgtctttgataactgcttcttacgccaaggctggggcaccagctgcctgattaattaaacaggccccttttcctttgtcgatatcatgtaattagttatgtcacgcttacattcacgccctcctcccacatccgctctaaccgaaaaggaaggagttagacaacctgaagtctaggtccctatttatttttttatagttatgttagtattaagaacgttatttatatttcaaatttttcttttttttctgtacaaacgcgtgtacgcatgtaacgggcagacggccggccataacttcgtataatgtatgctatacgaagttatggcaacggttcatcatctcatggatctgcacatgaacaaacaccagagtcaaacgacgttgaaattgaggctactgcgccaattgatgacaatacagacgatgataacaaaccgaagttatctgatgtagaaaaggattagagatgctaagagatagtgatgatatttcataaataatgtaattctatatatgttaattaccttttttgcgaggcatatttatggtgaaggataagttttgaccatcaaagaaggttaatgtggctgtggtttcagggtccataaagcttttcaattcatcttttttttttttgttcttttttttgattccggtttctttgaaatttttttgattcggtaatctccgagcagaaggaagaacgaaggaaggagcacagacttagattggtatatatacgcatatgtggtgttgaagaaacatgaaattgcccagtattcttaacccaactgcacagaacaaaaacctgcaggaaacgaagataaatcatgtcgaaagctacatataaggaacgtgctgctactcatcctagtcctgttgctgccaagctatttaatatcatgcacgaaaagcaaacaaacttgtgtgcttcattggatgttcgtaccaccaaggaattactggagttagttgaagcattaggtcccaaaatttgtttactaaaaacacatgtggatatcttgactgatttttccatggagggcacagttaagccgctaaaggcattatccgccaagtacaattttttactcttcgaagacagaaaatttgctgacattggtaatacagtcaaattgcagtactctgcgggtgtatacagaatagcagaatgggcagacattacgaatgcacacggtgtggtgggcccaggtattgttagcggtttgaagcaggcggcggaagaagtaacaaaggaacctagaggccttttgatgttagcagaattgtcatgcaagggctccctagctactggagaatatactaagggtactgttgacattgcgaagagcgacaaagattttgttatcggctttattgctcaaagagacatgggtggaagagatgaaggttacgattggttgattatgacacgcaggttacgattggttgattatgacacgc

SEQ ID NO: 27 - DNA, 4824 bp, synthetic construct
  misc_feature 1..4824: note = Rhizopus delemar GA integration construct
  source 1..4824: mol_type = other DNA
ggccgctccatggagggcacagttaagccgctaaaggcattatccgccaagtacaattttttactcttcgaagacagaaaatttgctgacattggtaatacagtcaaattgcagtactctgcgggtgtatacagaatagcagaatgggcagacattacgaatgcacacggtgtggtgggcccaggtattgttagcggtttgaagcaggcggcggaagaagtaacaaaggaacctagaggccttttgatgttagcagaattgtcatgcaagggctccctagctactggagaatatactaagggtactgttgacattgcgaagagcgacaaagattttgttatcggctttattgctcaaagagacatgggtggaagagatgaaggttacgattggttgattatgacacccggtgtgggtttagatgacaagggagacgcattgggtcaacagtatagaaccgtggatgatgtggtctctacaggatctgacattattattgttggaagaggactatttgcaaagggaagggatgctaaggtagagggtgaacgttacagaaaagcaggctgggaagcatatttgagaagatgcggccagcaaaactaaaaaactgtattataagtaaatgcatgtatactaaactcacaaattagagcttcaatttaattatatcagttattacccgggaatctcggtcgtaatgatttttataatgacgaaaaaaaaaaaattggaaagaaaaagcttcatggcctttataaaaaggaaccatccaatacctcgccagaaccaagtaacagtattttacggggcacaaatcaagaacaataagacaggactgtaaagatggacgcattgaactccaaagaacaacaagagttccaaaaagtagtggaacaaaagcaaatgaaggatttcatgcgtttgataacttcgtataatgtatgctatacgaagttatctcgagggccagaaaaaggaagtgtttccctccttcttgaattgatgttaccctcataaagcacgtggcctcttatcgagaaagaaattaccgtcgctcgtgatttgtttgcaaaaagaacaaaactgaaaaaacccagacacgctcgacttcctgtcttcctgttgattgcagcttccaatttcgtcacacaacaaggtcctagcgacggctcacaggttttgtaacaagcaatcgaaggttctggaatggcgggaaagggtttagtaccacatgctatgatgcccactgtgatctccagagcaaagttcgttcgatcgtactgttactctctctctttcaaacagaattgtccgaatcgtgtgacaacaacagcctgttctcacacactcttttcttctaaccaagggggtggtttagtttagtagaacctcgtgaaacttacatttacatatatataaacttgcataaattggtcaatgcaagaaatacatatttggtcttttctaattcgtagtttttcaagttcttagatgctttctttttctcttttttacagatcatcaaggaagtaattatctactttttacaagtctagaatgcagctgttcaacttgccattaaaggtttcattctttttggtcctatcatactttagtttgttggtgtcagccgcatctattccatcttcagcatctgtacaattagactcctacaattacgacggctctacattcagcggaaagatttacgtgaaaaatattgcgtacagcaaaaaagtaactgttatctatgccgacggatcagataactggaacaacaatggaaacactatcgctgccagttactctgcaccaatttcaggttctaactacgaatattggacattctcagcctccatcaatggcattaaggaattctacataaagtacgaagtttccggtaagacttactacgataacaacaattctgcaaactatcaagtatcaacatcaaaacctactaccaccaccgccacagctacaactacaactgcaccttcaacatctaccacaaccccaccatcttctagcgaaccagctacattcccaactggcaattctactatttctagttggatcaaaaaacaagagggtatttccagattcgcaatgttgagaaacataaatccaccaggatcagcaactggattcatcgcagcttctttgtccacagcggggccagattactactacgcatggaccagagatgctgctttgacaagtaacgttattgtttacgaatacaataccactttgtccggtaacaagactattcttaacgtcctaaaggattacgttacattctctgttaagactcagtctacatccacagtctgcaattgtttgggtgaaccaaagttcaacccagatggctctggatacacaggtgcctggggtcgtccacaaaacgatgggcctgccgagagagccactacatttatcctatttgctgactcataccttacacaaacaaaagatgcatcctacgtgactggaacattaaagcctgcaatcttcaaagacctggattacgttgtcaacgtgtggtctaacggctgtttcgatctatgggaagaggttaacggcgtgcacttctacactctaatggtcatgagaaagggtctgttgttaggtgcagattttgctaagagaaacggtgattctacacgtgcttctacctactcctcaacagcatcaactattgcgaacaagatttcttcattttgggtttcaagtaataactggatacaagtatctcaaagcgttacagggggtgtctcaaaaaagggtcttgatgtttctacattactggctgctaatcttgggtctgttgatgacggtttcttcacccctggttctgaaaagatcctcgctaccgccgtcgcggttgaggatagttttgcttcactctatcctataaacaaaaaccttccttcatacttaggaaacagtatcggtagatacccagaggatacatacaatggtaatggcaattcacagggaaatccatggttccttgctgttacagggtacgcagaactttactatagagctattaaggaatggatcggcaacggcggtgtgacagtttcctcaatctcattgccatttttcaaaaagtttgactccagcgcgacatctggtaaaaagtatactgtggggacttctgatttcaacaatttggctcaaaacattgccttagctgccgacagattcttatctaccgtacaactccatgcacataacaatggtagtttggcagaggaatttgatagaactacaggactctctacaggtgcgagagatttaacttggtcacatgcaagtttaattacagcctcttacgcaaaggctggtgctcctgctgcataattaattaatttaccagcttactatccttcttgaaaatatgcactctatatcttttagttcttaattgcaacacatagatttgctgtataacgaattttatgctatttttttaatttggagttcggtgatgaaagtgtcacagcgaatttcctcacatgtagggaccgaattgtttacaagttctctgtaccaccatggagacatcaaagattgaaaatctatggaaagatatggacggtagcaacaagaatatagcacgagccgcggagttcatttcgttacttttgatatcgctcacaactattgcgaagcgcttcagtgaaaaaatcataaggaaaagttgtaaatattattggtagtattcgtttggtaaagtagagggggtaatttttcccctttattttgttcatacattcttaaattgctttgcctctccttttggaaagctatacttcggagcactgttgagcgaaggctcaggccggcagcacgcagcacgctgtatttacgtatttaattttatatatttgtgcatacactactagggaagacttgaaaaaaacctaggaaatgaaaaaacgacacaggaagtcccgtatttactattttttccttccttttgatggggcagggcggaaatagaggataggataagcctactgcttagctgtttccgtctctacttcggtagttgtctcaattgtcgtttcagtattacctttagagccgctagacgatggttgagctatttgttgagggaaaactaagttcatgtaacacacgcataacccgattaaactcatgaatagcttgattgcaggaggctggtccattggagatggtgccttattttccttataggcaacgatgatgtcttcgtcggtgttcaggtagtagtgtacactctgaatcagggagaaccaggcaatgaacttgttcctcaagaaaatagcggccataggcatggattggttaaccacaccagatatgcttggtgtggcagaatatagtccttttggtggcgcaattttcttgtacctgtggtagaaagggagcggttgaactgttagtatatattggcaatatcagcaaatttgaaagaaaattgtcggtgaaaaacatacgaaacacaaaggtcgggccttgcaacgttattcaaagtcattgtttagttgaggaggtagcagcggagtatatgtattccttttttttgcctatggatgttgtaccatgcccattctgctcaagcttttgttaaaattatttttcagtattttttcttccatgttgcgcgttacgagaacagaagcgacagataaccgcaatcatacaactagcgctactgcggggtgtaaaaagcacaagaactaagccaagatcacaacagttatcgataaaatagcagtgtttgcatggccattgagaaggacaacattggcgtgcggcatg

SEQ ID NO: 28 - DNA, 5264 bp, synthetic construct
  misc_feature 1..5264: note = Rhizopus delemar GA integration construct
  source 1..5264: mol_type = other DNA
ctaaattcggccttgctcagagactcctggattttggctaacaacgcagtcccttcgatgcatatagctaggccacaaattatgccaataacggtccatgggttgatgttttcttgaattctttcgtttttcatgctatttgcgtcttcccaagtcccagcgttccagtattcatactgcgcgttagagtggtagccataagagccggcatattggtaattttcagtattaacgttagaacgtggtgaatacgatgtggtccagccttgcctcgttgtgtcatatacgatctttttctttgggtcacaaagaatatcatatgcttgagagatgactttaaatctatgtagtttttcgcttgatgttagcagcagcggtgatttactatcactgttggtaaccttttctgagctaaatatttgaatgttatcggaatggtcagggtggtacaattttacataacgatgatattttttttttaacgacttcttgtccagtttaggatttccagatccggcctttggaatgccaaaaatatcatagggagttggatctgccaactcaggccattgttcatcccttatcgtaagttttctattgccatttttatcgttcgctgtagcatacttagctataaaagtgatttgtgggggacacttttctacacatgataagtgccacttgaataaaaatgggtatacgaacttatggtgtagcataacaaatatattgcaagtagtgacctatggtgtgtagatatacgtacagttagttacgagcctaaagacacaacgtgtttgttaattatactgtcgctgtaatatcttctcttccattatcaccggtcattccttgcaggggcggtagtacccggagaccctgaacttttctttttttttttgcgaaattaaaaagttcattttcaattcgacaatgagatctacaagccattgttttatgttgatgagagccagcttaaagagttctcgagatctcccgagtttatcattatcaatactgccatttcaaagaatacgtaaataattaatagtagtgattttcctaactttatttagtcaaaaaattggccttttaattctgctgtaacccgtacatgcccaaaatagggggcgggttacacagaatatataacatcataggtgtctgggtgaacagtttattcctggcatccactaaatataatggagcccgctttttttaagctggcatccagaaaaaaaaagaatcccagcaccaaaatattgttttcttcaccaaccatcagttcataggtccattctcttagcgcaactacacagaacaggggcacaaacaggcaaaaaacgggcacaacctcaatggagtgatgcaacctgcttggagtaaatgatgacacaaggcaattgacctacgcatgtatctatctcattttcttacaccttctattaccttctgctctctctgatttggaaaaagctgaaaaaaaaggttgaaaccagttccctgaaattattcccctatttgactaataagtatataaagacggtaggtattgattgtaattctgtaaatctatttcttaaacttcttaaattctacttttatagttagtcttttttttagtttaaaacaccaagaacttagtttcgaataaacacacataaacaaacaaatctagaatgcagttattcaacttaccacttaaggtatctttctttctagtcttatcttacttttcattgttagtatcagctgcctctataccaagttcagcatccgtacaactagattcatacaattacgacggttcaacattctcaggaaagatatacgtgaaaaatattgcttacagcaaaaaggttactgtgatttacgcagatgggtcagacaactggaataacaatggaaacacaattgctgcttcctattctgcccctatttctggatctaactacgaatactggactttttcagcgagtataaacggaattaaggaattctatatcaaatatgaagtctctggtaagacctactacgataacaacaactccgcaaactaccaagttagcacatcaaagccaaccacaacaactgctactgcgacaactacaaccgcaccaagcacttctactacaacacctcctagttcatctgagccagcaactttcccaactggtaattccactatttcttcttggatcaaaaaacaagagggtatctcaagattcgccatgcttagaaatatcaatcctccaggctctgcaacaggattcattgcagcatctttatcaactgcggggccagactactactacgcctggactagagatgcagctttgacatcaaatgtgattgtttatgaatacaacacaactttgtccggtaacaagacaatcttgaacgtcttgaaggattatgtgacattctctgtcaagactcaatctacatcaacagtttgtaactgtctcggcgaaccaaagttcaaccctgatggtagtggttacactggtgcttggggtagaccacaaaacgatggtccagcagagagagctacaactttcatcttgtttgctgactcttacctaacacaaaccaaggatgcaagctacgttactggaacactaaagcctgcaatctttaaagacctggactatgttgtaaacgtttggtcaaatggctgcttcgatctatgggaggaagtgaacggtgttcacttctacacattaatggtcatgagaaagggactcttgcttggtgcagactttgctaagagaaacggtgattctacacgtgcctccacttactcctccacagcttcaaccattgccaacaaaatctcttctttctgggtcagctcaaataactggattcaagtttctcaatcagttactggtggtgtttctaaaaagggcctggatgtgtcaaccttgcttgctgccaatttgggcagtgttgatgacgggttcttcaccccaggttctgaaaagatcctcgccaccgcagttgccgttgaagattcatttgctagtttatacccaatcaacaaaaatctaccatcataccttggaaattcaatcggtagatatccagaggatacatacaacggtaatggaaactctcagggtaacccttggtttcttgcagttacagggtacgctgaactgtactacagagcgattaaggaatggattggtaatggcggcgtaactgttagttctatttctctacctttcttcaaaaagttcgatagttctgcaacatctggtaaaaagtacacagtcggcacttccgattttaacaatttagctcagaacatagcactggcagctgatcgtttcttgagtacagtccaattgcatgcccataacaacggtagtttggctgaagagtttgatagaaccaccggtttatcaaccggcgccagagatttaacatggtcccatgcgtctttgataactgcttcttacgccaaggctggggcaccagctgcctgattaattaaacaggccccttttcctttgtcgatatcatgtaattagttatgtcacgcttacattcacgccctcctcccacatccgctctaaccgaaaaggaaggagttagacaacctgaagtctaggtccctatttatttttttatagttatgttagtattaagaacgttatttatatttcaaatttttcttttttttctgtacaaacgcgtgtacgcatgtaacgggcagacggccggccataacttcgtataatgtatgctatacgaagttatccttacatcacacccaatcccccacaagtgatcccccacacaccatagcttcaaaatgtttctactccttttttactcttccagattttctcggactccgcgcatcgccgtaccacttcaaaacacccaagcacagcatactaaatttcccctctttcttcctctagggtggcgttaattacccgtactaaaggtttggaaaagaaaaaagagaccgcctcgtttctttttcttcgtcgaaaaaggcaataaaaatttttatcacgtttctttttcttgaaaaattttttttttgatttttttctctttcgatgacctcccattgatatttaagttaataaatggtcttcaatttctcaagtttcagtttcgtttttcttgttctattacaactttttttacttcttgctcattagaaagaaagcatagcaatctaatctaagttttaattacaaaatgccacaatcctgggaagaattggccgccgacaaacgtgcccgtttggctaaaaccattcctgacgaatggaaggttcaaactttgcctgccgaagattccgttattgatttcccaaagaagtccggtattttgtctgaggctgaattgaagattaccgaagcctctgctgctgatttggtctccaagttggccgctggtgagttgacttctgttgaagtcactttggctttttgtaagagagctgctattgctcaacaattaaccaactgtgctcacgaattcttcccagatgctgctttagctcaagctagagaattagatgaatactacgctaagcataagagaccagttggtccattacacggtttaccaatctctttaaaggaccaattgcgtgttaagggttacgaaacctccatgggttacatttcctggttaaacaaatacgatgaaggtgattccgtcttaaccaccatgttgagaaaagctggtgctgttttctacgttaagacctctgtcccacaaaccttgatggtctgtgaaaccgtcaacaacatcattggtagaactgtcaatccaagaaacaaaaattggtcctgtggtggttcttctggtggtgaaggtgctattgttggtattagaggtggtgttattggtgtcggtactgacattggtggttccattagagtcccagctgctttcaactttttatacggtttgagaccatctcacggtagattgccatatgctaaaatggctaactctatggaaggtcaagaaaccgttcactccgtcgttggtcctatcactcactccgtcgaagacttgagattgttcaccaaatctgtcttgggtcaagaaccttggaagtacgactctaaggtcatccccatgccatggagacaatctgaatctgacatcattgcctctaagattaagaatggtggtttgaacattggttattacaatttcgacggtaacgtcttgccacacccaccaattttacgtggtgtcgaaactaccgttgccgctttggc

SEQ ID NO: 29 - DNA, 5026 bp, synthetic construct
  misc_feature 1..5026: note = Rhizopus delemar GA integration construct
  source 1..5026: mol_type = other DNA
ggccgcgaaggtgctattgttggtattagaggtggtgttattggtgtcggtactgacattggtggttccattagagtcccagctgctttcaactttttatacggtttgagaccatctcacggtagattgccatatgctaaaatggctaactctatggaaggtcaagaaaccgttcactccgtcgttggtcctatcactcactccgtcgaagacttgagattgttcaccaaatctgtcttgggtcaagaaccttggaagtacgactctaaggtcatcccaatgccatggagacaatctgaatctgacatcattgcctctaagattaagaatggtggtttgaacattggttattacaatttcgacggtaacgtcttgccacacccaccaattttacgtggtgtcgaaactaccgttgccgctttggccaaggctggtcacaccgttactccatggactccatacaagcatgatttcggtcatgacttgatttcccacatctatgctgctgatggttctgccgacgtcatgagagacatttctgcctctggtgagccagccatccctaacattaaggacttgttgaacccaaatattaaggctgttaacatgaacgaattgtgggacactcatttacaaaagtggaactatcaaatggaatacttggaaaagtggcgtgaagctgaagaaaaagctggtaaggaattggacgctattatcgctccaattactcctaccgccgctgtcagacacgatcaattcagatactacggttacgcctccgttattaacttattggatttcacctctgttgtcgtcccagtcactttcgctgataagaatattgataagaagaacgaatcttttaaagctgtttccgaattggatgctttggttcaagaagaatacgacccagaggcttatcacggtgctcctgttgctgttcaagttattggtagaagattgtccgaagagagaactttggctatcgccgaagaagtcggtaaattgttgggtaacgtcgtcactccataagcgaatttcttatgatttatgatttttattattaaataagttataaaaaaaataagtgtatacaaattttaaagtgactcttaggttttaaaacgaaaattcttattcttgagtaactctttcctgtaggtcaggttgctttctcaggtatagcatgaggtcgctcttattgaccacacctctaccggcatgccgagcaaatgcctgcaaatcgctccccatttcacccaattgtagatatgctaactccagcaatgagttgatgaatctcggtgtgtattttatgtcctcagaggacaacacataacttcgtataatgtatgctatacgaagttatctcgagggccagaaaaaggaagtgtttccctccttcttgaattgatgttaccctcataaagcacgtggcctcttatcgagaaagaaattaccgtcgctcgtgatttgtttgcaaaaagaacaaaactgaaaaaacccagacacgctcgacttcctgtcttcctgttgattgcagcttccaatttcgtcacacaacaaggtcctagcgacggctcacaggttttgtaacaagcaatcgaaggttctggaatggcgggaaagggtttagtaccacatgctatgatgcccactgtgatctccagagcaaagttcgttcgatcgtactgttactctctctctttcaaacagaattgtccgaatcgtgtgacaacaacagcctgttctcacacactcttttcttctaaccaagggggtggtttagtttagtagaacctcgtgaaacttacatttacatatatataaacttgcataaattggtcaatgcaagaaatacatatttggtcttttctaattcgtagtttttcaagttcttagatgctttctttttctcttttttacagatcatcaaggaagtaattatctactttttacaagtctagaatgcagctgttcaacttgccattaaaggtttcattctttttggtcctatcatactttagtttgttggtgtcagccgcatctattccatcttcagcatctgtacaattagactcctacaattacgacggctctacattcagcggaaagatttacgtgaaaaatattgcgtacagcaaaaaagtaactgttatctatgccgacggatcagataactggaacaacaatggaaacactatcgctgccagttactctgcaccaatttcaggttctaactacgaatattggacattctcagcctccatcaatggcattaaggaattctacataaagtacgaagtttccggtaagacttactacgataacaacaattctgcaaactatcaagtatcaacatcaaaacctactaccaccaccgccacagctacaactacaactgcaccttcaacatctaccacaaccccaccatcttctagcgaaccagctacattcccaactggcaattctactatttctagttggatcaaaaaacaagagggtatttccagattcgcaatgttgagaaacataaatccaccaggatcagcaactggattcatcgcagcttctttgtccacagcggggccagattactactacgcatggaccagagatgctgctttgacaagtaacgttattgtttacgaatacaataccactttgtccggtaacaagactattcttaacgtcctaaaggattacgttacattctctgttaagactcagtctacatccacagtctgcaattgtttgggtgaaccaaagttcaacccagatggctctggatacacaggtgcctggggtcgtccacaaaacgatgggcctgccgagagagccactacatttatcctatttgctgactcataccttacacaaacaaaagatgcatcctacgtgactggaacattaaagcctgcaatcttcaaagacctggattacgttgtcaacgtgtggtctaacggctgtttcgatctatgggaagaggttaacggcgtgcacttctacactctaatggtcatgagaaagggtctgttgttaggtgcagattttgctaagagaaacggtgattctacacgtgcttctacctactcctcaacagcatcaactattgcgaacaagatttcttcattttgggtttcaagtaataactggatacaagtatctcaaagcgttacagggggtgtctcaaaaaagggtcttgatgtttctacattactggctgctaatcttgggtctgttgatgacggtttcttcacccctggttctgaaaagatcctcgctaccgccgtcgcggttgaggatagttttgcttcactctatcctataaacaaaaaccttccttcatacttaggaaacagtatcggtagatacccagaggatacatacaatggtaatggcaattcacagggaaatccatggttccttgctgttacagggtacgcagaactttactatagagctattaaggaatggatcggcaacggcggtgtgacagtttcctcaatctcattgccatttttcaaaaagtttgactccagcgcgacatctggtaaaaagtatactgtggggacttctgatttcaacaatttggctcaaaacattgccttagctgccgacagattcttatctaccgtacaactccatgcacataacaatggtagtttggcagaggaatttgatagaactacaggactctctacaggtgcgagagatttaacttggtcacatgcaagtttaattacagcctcttacgcaaaggctggtgctcctgctgcataattaattaatttaccagcttactatccttcttgaaaatatgcactctatatcttttagttcttaattgcaacacatagatttgctgtataacgaattttatgctatttttttaatttggagttcggtgatgaaagtgtcacagcgaatttcctcacatgtagggaccgaattgtttacaagttctctgtaccaccatggagacatcaaagattgaaaatctatggaaagatatggacggtagcaacaagaatatagcacgagccgcggagttcatttcgttacttttgatatcgctcacaactattgcgaagcgcttcagtgaaaaaatcataaggaaaagttgtaaatattattggtagtattcgtttggtaaagtagagggggtaatttttcccctttattttgttcatacattcttaaattgctttgcctctccttttggaaagctatacttcggagcactgttgagcgaaggctcaggccggcagcacgcagcacgctgtatttacgtatttaattttatatatttgtgcatacactactagggaagacttgaaaaaaacctaggaaatgaaaaaacgacacaggaagtcccgtatttactattttttccttccttttgatggggcagggcggaaatagaggataggataagcctactgcttagctgtttccgtctctacttcggtagttgtctcaattgtcgtttcagtattacctttagagccgctagacgatggttgagctatttgttgagggaaaactaagttcatgtaacacacgcataacccgattaaactcatgaatagcttgattgcaggaggctggtccattggagatggtgccttattttccttataggcaacgatgatgtcttcgtcggtgttcaggtagtagtgtacactctgaatcagggagaaccaggcaatgaacttgttcctcaagaaaatagcggccataggcatggattggttaaccacaccagatatgcttggtgtggcagaatatagtccttttggtggcgcaattttcttgtacctgtggtagaaagggagcggttgaactgttagtatatattggcaatatcagcaaatttgaaagaaaattgtcggtgaaaaacatacgaaacacaaaggtcgggccttgcaacgttattcaaagtcattgtttagttgaggaggtagcagcggagtatatgtattccttttttttgcctatggatgttgtaccatgcccattctga